European Patent Application EP 4 545 566 A2, published April 30, 2025. Title: SELECTIVE MODULATION OF TRANSFORMING GROWTH FACTOR BETA SUPERFAMILY SIGNALING VIA MULTI-SPECIFIC ANTIBODIES. Applicant: THE BRIGHAM AND WOMEN'S HOSPITAL, INC. Application WO PCT/US2021/020291, filed March 1, 2021. The sequence listing filed with the application follows.

SEQUENCE LISTING (613 sequences)

SEQ ID NO: 1 - protein, 8 aa, synthetic construct
  REGION 1..8: note = Description of Artificial Sequence: Synthetic peptide
KLGDKYAS

SEQ ID NO: 2 - protein, 11 aa, synthetic construct
  REGION 1..11: note = Description of Artificial Sequence: Synthetic peptide
LVIYQDSKRPS

SEQ ID NO: 3 - protein, 8 aa, synthetic construct
  REGION 1..8: note = Description of Artificial Sequence: Synthetic peptide
QAWDSSTA

SEQ ID NO: 4 - protein, 11 aa, synthetic construct
  REGION 1..11: note = Description of Artificial Sequence: Synthetic peptide
GSISSDDYYWS

SEQ ID NO: 5 - protein, 13 aa, synthetic construct
  REGION 1..13: note = Description of Artificial Sequence: Synthetic peptide
WIGYIYYSGITYY

SEQ ID NO: 6 - protein, 16 aa, synthetic construct
  REGION 1..16: note = Description of Artificial Sequence: Synthetic peptide
REGCNDGVCYNGVFDY

SEQ ID NO: 7 - protein, 11 aa, synthetic construct
  REGION 1..11: note = Description of Artificial Sequence: Synthetic peptide
SSDVGTYNYVS

SEQ ID NO: 8 - protein, 11 aa, synthetic construct
  REGION 1..11: note = Description of Artificial Sequence: Synthetic peptide
LMIYDVSKRPS

SEQ ID NO: 9 - protein, 9 aa, synthetic construct
  REGION 1..9: note = Description of Artificial Sequence: Synthetic peptide
YSYTTSSTW

SEQ ID NO: 10 - protein, 11 aa, synthetic construct
  REGION 1..11: note = Description of Artificial Sequence: Synthetic peptide
DSIGSGDYYWS

SEQ ID NO: 11 - protein, 13 aa, synthetic construct
  REGION 1..13: note = Description of Artificial Sequence: Synthetic peptide
WIGYSYHTGSTDY

SEQ ID NO: 12 - protein, 9 aa, synthetic construct
  REGION 1..9: note = Description of Artificial Sequence: Synthetic peptide
RDYYGYLGY

SEQ ID NO: 13 - protein, 8 aa, synthetic construct
  REGION 1..8: note = Description of Artificial Sequence: Synthetic peptide
QSISSYLN

SEQ ID NO: 14 - protein, 11 aa, synthetic construct
  REGION 1..11: note = Description of Artificial Sequence: Synthetic peptide
LLIYAASSLQS

SEQ ID NO: 15 - protein, 8 aa, synthetic construct
  REGION 1..8: note = Description of Artificial Sequence: Synthetic peptide
QQSYSTPR

SEQ ID NO: 16 - protein, 11 aa, synthetic construct
  REGION 1..11: note = Description of Artificial Sequence: Synthetic peptide
GSISSDDYYWS

SEQ ID NO: 17 - protein, 13 aa, synthetic construct
  REGION 1..13: note = Description of Artificial Sequence: Synthetic peptide
WIGYIYYSGITYY

SEQ ID NO: 18 - protein, 16 aa, synthetic construct
  REGION 1..16: note = Description of Artificial Sequence: Synthetic peptide
REGCNDGVCYNGVFDY

SEQ ID NO: 19 - protein, 10 aa, synthetic construct
  REGION 1..10: note = Description of Artificial Sequence: Synthetic peptide
SSNIGGNTVN

SEQ ID NO: 20 - protein, 11 aa, synthetic construct
  REGION 1..11: note = Description of Artificial Sequence: Synthetic peptide
LLIYGDDLRPS

SEQ ID NO: 21 - protein, 10 aa, synthetic construct
  REGION 1..10: note = Description of Artificial Sequence: Synthetic peptide
AAWDDSLNAY

SEQ ID NO: 22 - protein, 10 aa, synthetic construct
  REGION 1..10: note = Description of Artificial Sequence: Synthetic peptide
FTFSNYAMHS

SEQ ID NO: 23 - protein, 14 aa, synthetic construct
  REGION 1..14: note = Description of Artificial Sequence: Synthetic peptide
WVAVISYDGSNKYY

SEQ ID NO: 24 - protein, 13 aa, synthetic construct
  REGION 1..13: note = Description of Artificial Sequence: Synthetic peptide
RVRYYGSGSPIGY

SEQ ID NO: 25 - protein, 11 aa, synthetic construct
  REGION 1..11: note = Description of Artificial Sequence: Synthetic peptide
SSDVGGYKSVS

SEQ ID NO: 26 - protein, 11 aa, synthetic construct
  REGION 1..11: note = Description of Artificial Sequence: Synthetic peptide
LMIYDVSNRPS

SEQ ID NO: 27 - protein, 10 aa, synthetic construct
  REGION 1..10: note = Description of Artificial Sequence: Synthetic peptide
SSYTSSSSLW

SEQ ID NO: 28 - protein, 9 aa, synthetic construct
  REGION 1..9: note = Description of Artificial Sequence: Synthetic peptide
GTFSSYAIS

SEQ ID NO: 29 - protein, 14 aa, synthetic construct
  REGION 1..14: note = Description of Artificial Sequence: Synthetic peptide
WMGRIIPILGIANY

SEQ ID NO: 30 - protein, 9 aa, synthetic construct
  REGION 1..9: note = Description of Artificial Sequence: Synthetic peptide
TDLWGVGAD

SEQ ID NO: 31 - protein, 11 aa, synthetic construct
  REGION 1..11: note = Description of Artificial Sequence: Synthetic peptide
NTDIGYYNYVS

SEQ ID NO: 32 - protein, 11 aa, synthetic construct
  REGION 1..11: note = Description of Artificial Sequence: Synthetic peptide
LLIFEVDNRPS

SEQ ID NO: 33 - protein, 9 aa, synthetic construct
  REGION 1..9: note = Description of Artificial Sequence: Synthetic peptide
SSYSTYNIL

SEQ ID NO: 34 - protein, 9 aa, synthetic construct
  REGION 1..9: note = Description of Artificial Sequence: Synthetic peptide
YTFTGYYMH

SEQ ID NO: 35 - protein, 15 aa, synthetic construct
  REGION 1..15: note = Description of Artificial Sequence: Synthetic peptide
WMGRINPNSGGTNYA

SEQ ID NO: 36 - protein, 14 aa, synthetic construct
  REGION 1..14: note = Description of Artificial Sequence: Synthetic peptide
RDPTYYDILTGPEY

SEQ ID NO: 37 - protein, 8 aa, synthetic construct
  REGION 1..8: note = Description of Artificial Sequence: Synthetic peptide
QSVSSNLA

SEQ ID NO: 38 - protein, 11 aa, synthetic construct
  REGION 1..11: note = Description of Artificial Sequence: Synthetic peptide
LLIYGASSRAT

SEQ ID NO: 39 - protein, 8 aa, synthetic construct
  REGION 1..8: note = Description of Artificial Sequence: Synthetic peptide
QQYIYSPY

SEQ ID NO: 40 - protein, 9 aa, synthetic construct
  REGION 1..9: note = Description of Artificial Sequence: Synthetic peptide
YNFAGYYVH

SEQ ID NO: 41 - protein, 15 aa, synthetic construct
  REGION 1..15: note = Description of Artificial Sequence: Synthetic peptide
WMGWINPNSGGTDYA

SEQ ID NO: 42 - protein, 8 aa, synthetic construct
  REGION 1..8: note = Description of Artificial Sequence: Synthetic peptide
RNLQFFRP

SEQ ID NO: 43 - protein, 8 aa, synthetic construct
  REGION 1..8: note = Description of Artificial Sequence: Synthetic peptide
NIGSKNVH

SEQ ID NO: 44 - protein, 11 aa, synthetic construct
  REGION 1..11: note = Description of Artificial Sequence: Synthetic peptide
LVIYDDSDRPS

SEQ ID NO: 45 - protein, 9 aa, synthetic construct
  REGION 1..9: note = Description of Artificial Sequence: Synthetic peptide
QAWDSSTAV

SEQ ID NO: 46 - protein, 11 aa, synthetic construct
  REGION 1..11: note = Description of Artificial Sequence: Synthetic peptide
GSISSSSYYWG

SEQ ID NO: 47 - protein, 13 aa, synthetic construct
  REGION 1..13: note = Description of Artificial Sequence: Synthetic peptide
WIGSIYYSGSTYY

SEQ ID NO: 48 - protein, 11 aa, synthetic construct
  REGION 1..11: note = Description of Artificial Sequence: Synthetic peptide
RQVGPVLKSVS

SEQ ID NO: 49 - protein, 9 aa, synthetic construct
  REGION 1..9: note = Description of Artificial Sequence: Synthetic peptide
FTFSSYAMS

SEQ ID NO: 50 - protein, 14 aa, synthetic construct
  REGION 1..14: note = Description of Artificial Sequence: Synthetic peptide
WVSAISGSGGSTYY

SEQ ID NO: 51 - protein, 8 aa, synthetic construct
  REGION 1..8: note = Description of Artificial Sequence: Synthetic peptide
KSASFFDY

SEQ ID NO: 52 - protein, 9 aa, synthetic construct
  REGION 1..9: note = Description of Artificial Sequence: Synthetic peptide
QSVSSSYLA

SEQ ID NO: 53 - protein, 11 aa, synthetic construct
  REGION 1..11: note = Description of Artificial Sequence: Synthetic peptide
LLIYGASSRAT

SEQ ID NO: 54 - protein, 8 aa, synthetic construct
  REGION 1..8: note = Description of Artificial Sequence: Synthetic peptide
QQHFRWPW

SEQ ID NO: 55 - protein, 10 aa, synthetic construct
  REGION 1..10: note = Description of Artificial Sequence: Synthetic peptide
SSNIGSNTVN

SEQ ID NO: 56 - protein, 11 aa, synthetic construct
  REGION 1..11: note = Description of Artificial Sequence: Synthetic peptide
LLIYSNNQRPS

SEQ ID NO: 57 - protein, 10 aa, synthetic construct
  REGION 1..10: note = Description of Artificial Sequence: Synthetic peptide
AAWDDSLNGV

SEQ ID NO: 58 - protein, 11 aa, synthetic construct
  REGION 1..11: note = Description of Artificial Sequence: Synthetic peptide
ASISSGGYYWS

SEQ ID NO: 59 - protein, 13 aa, synthetic construct
  REGION 1..13: note = Description of Artificial Sequence: Synthetic peptide
WIGYSYYSGSTYY

SEQ ID NO: 60 - protein, 8 aa, synthetic construct
  REGION 1..8: note = Description of Artificial Sequence: Synthetic peptide
RGGVRFDL

SEQ ID NO: 61 - protein, 8 aa, synthetic construct
  REGION 1..8: note = Description of Artificial Sequence: Synthetic peptide
ALPKKYAY

SEQ ID NO: 62 - protein, 11 aa, synthetic construct
  REGION 1..11: note = Description of Artificial Sequence: Synthetic peptide
LVIYEDSKRPS

SEQ ID NO: 63 - protein, 9 aa, synthetic construct
  REGION 1..9: note = Description of Artificial Sequence: Synthetic peptide
YSTDSSGNP

SEQ ID NO: 64 - protein, 9 aa, synthetic construct
  REGION 1..9: note = Description of Artificial Sequence: Synthetic peptide
FTFSSYAMS

SEQ ID NO: 65 - protein, 14 aa, synthetic construct
  REGION 1..14: note = Description of Artificial Sequence: Synthetic peptide
WVSAISGSGGSTYY

SEQ ID NO: 66 - protein, 24 aa, synthetic construct
  REGION 1..24: note = Description of Artificial Sequence: Synthetic peptide
KIPWGDYDFWSGYYTRPGHSGMDV

SEQ ID NO: 67 - protein, 11 aa, synthetic construct
  REGION 1..11: note = Description of Artificial Sequence: Synthetic peptide
SSNIGAGYDVH

SEQ ID NO: 68 - protein, 11 aa, synthetic construct
  REGION 1..11: note = Description of Artificial Sequence: Synthetic peptide
LLIFDSSNRPS

SEQ ID NO: 69 - protein, 11 aa, synthetic construct
  REGION 1..11: note = Description of Artificial Sequence: Synthetic peptide
QSYDFRLSGSM

SEQ ID NO: 70 - protein, 9 aa, synthetic construct
  REGION 1..9: note = Description of Artificial Sequence: Synthetic peptide
FTFRAYPMS

SEQ ID NO: 71 - protein, 12 aa, synthetic construct
  REGION 1..12: note = Description of Artificial Sequence: Synthetic peptide
WVSSITSSGSYY

SEQ ID NO: 72 - protein, 9 aa, synthetic construct
  REGION 1..9: note = Description of Artificial Sequence: Synthetic peptide
RVGVTDFDY

SEQ ID NO: 73 - protein, 10 aa, synthetic construct
  REGION 1..10: note = Description of Artificial Sequence: Synthetic peptide
SSNIGTNYVY

SEQ ID NO: 74 - protein, 11 aa, synthetic construct
  REGION 1..11: note = Description of Artificial Sequence: Synthetic peptide
LLIYRNNQRPS

SEQ ID NO: 75 - protein, 10 aa, synthetic construct
  REGION 1..10: note = Description of Artificial Sequence: Synthetic peptide
AAWDDSLSGW

SEQ ID NO: 76 - protein, 9 aa, synthetic construct
  REGION 1..9: note = Description of Artificial Sequence: Synthetic peptide
FTFSSYAMS

SEQ ID NO: 77 - protein, 15 aa, synthetic construct
  REGION 1..15: note = Description of Artificial Sequence: Synthetic peptide
WVSAISGSGGSTYYA

SEQ ID NO: 78 - protein, 13 aa, synthetic construct
  REGION 1..13: note = Description of Artificial Sequence: Synthetic peptide
AKSIRTGSGYFDY

SEQ ID NO: 79 - protein, 10 aa, synthetic construct
  REGION 1..10: note = Description of Artificial Sequence: Synthetic peptide
SSNIGSNYVY

SEQ ID NO: 80 - protein, 11 aa, synthetic construct
  REGION 1..11: note = Description of Artificial Sequence: Synthetic peptide
LLIYRNNQRPS

SEQ ID NO: 81 - protein, 10 aa, synthetic construct
  REGION 1..10: note = Description of Artificial Sequence: Synthetic peptide
AAWDDSLSGW

SEQ ID NO: 82 - protein, 9 aa, synthetic construct
  REGION 1..9: note = Description of Artificial Sequence: Synthetic peptide
YTFTSYYMH

SEQ ID NO: 83 - protein, 15 aa, synthetic construct
  REGION 1..15: note = Description of Artificial Sequence: Synthetic peptide
WMGIINPSGGSTSYA

SEQ ID NO: 84 - protein, 14 aa, synthetic construct
  REGION 1..14: note = Description of Artificial Sequence: Synthetic peptide
RDLLLYGRGGGFQH

SEQ ID NO: 85 - protein, 8 aa, synthetic construct
  REGION 1..8: note = Description of Artificial Sequence: Synthetic peptide
SLRSYYAS

SEQ ID NO: 86 - protein, 11 aa, synthetic construct
  REGION 1..11: note = Description of Artificial Sequence: Synthetic peptide
LVIYGKNNRPS

SEQ ID NO: 87 - protein, 11 aa, synthetic construct
  REGION 1..11: note = Description of Artificial Sequence: Synthetic peptide
NSRDNSGKHLW

SEQ ID NO: 88 - protein, 9 aa, synthetic construct
  REGION 1..9: note = Description of Artificial Sequence: Synthetic peptide
FTFDDYGMS

SEQ ID NO: 89 - protein, 14 aa, synthetic construct
  REGION 1..14: note = Description of Artificial Sequence: Synthetic peptide
WVSGINWNGGSTGY

SEQ ID NO: 90 - protein, 7 aa, synthetic construct
  REGION 1..7: note = Description of Artificial Sequence: Synthetic peptide
RKSTGDY

SEQ ID NO: 91 - protein, 11 aa, synthetic construct
  REGION 1..11: note = Description of Artificial Sequence: Synthetic peptide
SSNIGAGYDVH

SEQ ID NO: 92 - protein, 11 aa, synthetic construct
  REGION 1..11: note = Description of Artificial Sequence: Synthetic peptide
LLIYGNSNRPS

SEQ ID NO: 93 - protein, 12 aa, synthetic construct
  REGION 1..12: note = Description of Artificial Sequence: Synthetic peptide
AAWDDSLNGPRM

SEQ ID NO: 94 - protein, 9 aa, synthetic construct
  REGION 1..9: note = Description of Artificial Sequence: Synthetic peptide
FTFSDYYMS

SEQ ID NO: 95 - protein, 14 aa, synthetic construct
  REGION 1..14: note = Description of Artificial Sequence: Synthetic peptide
WVSYISSSSSYTNY

SEQ ID NO: 96 - protein, 10 aa, synthetic construct
  REGION 1..10: note = Description of Artificial Sequence: Synthetic peptide
RVNYYYGMDV

SEQ ID NO: 97 - protein, 8 aa, synthetic construct
  REGION 1..8: note = Description of Artificial Sequence: Synthetic peptide
SLRKYYAS

SEQ ID NO: 98 - protein, 11 aa, synthetic construct
  REGION 1..11: note = Description of Artificial Sequence: Synthetic peptide
LVIYGKNKRPS

SEQ ID NO: 99 - protein, 10 aa, synthetic construct
  REGION 1..10: note = Description of Artificial Sequence: Synthetic peptide
NSWDSSGNHV

SEQ ID NO: 100 - protein, 11 aa, synthetic construct
  REGION 1..11: note = Description of Artificial Sequence: Synthetic peptide
GSISSGGYYWS

SEQ ID NO: 101 - protein, 13 aa, synthetic construct
  REGION 1..13: note = Description of Artificial Sequence: Synthetic peptide
WIGYIYYSGSTYY

SEQ ID NO: 102 - protein, 10 aa, synthetic construct
  REGION 1..10: note = Description of Artificial Sequence: Synthetic peptide
REEVGDWFDP

SEQ ID NO: 103 - protein, 6 aa, synthetic construct
  REGION 1..6: note = Description of Artificial Sequence: Synthetic peptide
GGGGSG

SEQ ID NO: 104 - protein, 9 aa, synthetic construct
  REGION 1..9: note = Description of Artificial Sequence: Synthetic peptide
GGGGSGGGS

SEQ ID NO: 105 - protein, 14 aa, synthetic construct
  REGION 1..14: note = Description of Artificial Sequence: Synthetic peptide
EGKSSGSGSDSKAS

SEQ ID NO: 106 - protein, 14 aa, synthetic construct
  REGION 1..14: note = Description of Artificial Sequence: Synthetic peptide
EGKSSGSGSESKAS

SEQ ID NO: 107 - protein, 27 aa, synthetic construct
  REGION 1..27: note = Description of Artificial Sequence: Synthetic peptide
SGGGGSGGGGSSGSGGGGDGGGGSGGT

SEQ ID NO: 108 - protein, 34 aa, synthetic construct
  REGION 1..34: note = Description of Artificial Sequence: Synthetic polypeptide
SGGSGGGGSSGGGGSGGGGSSGGGGDGGGGSGGT

SEQ ID NO: 109 - protein, 11 aa, synthetic construct
  REGION 1..11: note = Description of Artificial Sequence: Synthetic peptide
QGDSLRKYYAS

SEQ ID NO: 110 - protein, 11 aa, synthetic construct
  REGION 1..11: note = Description of Artificial Sequence: Synthetic peptide
LVIYGKSKRPS

SEQ ID NO: 111 - protein, 11 aa, synthetic construct
  REGION 1..11: note = Description of Artificial Sequence: Synthetic peptide
NSWDSSGNHVV

SEQ ID NO: 112 - protein, 12 aa, synthetic construct
  REGION 1..12: note = Description of Artificial Sequence: Synthetic peptide
GGSISSGGYYWS

SEQ ID NO: 113 - protein, 13 aa, synthetic construct
  REGION 1..13: note = Description of Artificial Sequence: Synthetic peptide
WIGYIYYSGSTYY

SEQ ID NO: 114 - protein, 10 aa, synthetic construct
  REGION 1..10: note = Description of Artificial Sequence: Synthetic peptide
REEVGDWFDP

SEQ ID NO: 115 - protein, 14 aa, synthetic construct
  REGION 1..14: note = Description of Artificial Sequence: Synthetic peptide
TLHSGINVATYRIY

SEQ ID NO: 116 - protein, 11 aa, synthetic construct
  REGION 1..11: note = Description of Artificial Sequence: Synthetic peptide
YKSDLDKHQGS

SEQ ID NO: 117 - protein, 9 aa, synthetic construct
  REGION 1..9: note = Description of Artificial Sequence: Synthetic peptide
LIWHDYVWY

SEQ ID NO: 118 - protein, 14 aa, synthetic construct
  REGION 1..14: note = Description of Artificial Sequence: Synthetic peptide
CAASGFTFDDYAMH

SEQ ID NO: 119 - protein, 14 aa, synthetic construct
  REGION 1..14: note = Description of Artificial Sequence: Synthetic peptide
WVSGISWNSGSIGY

SEQ ID NO: 120 - protein, 16 aa, synthetic construct
  REGION 1..16: note = Description of Artificial Sequence: Synthetic peptide
KGGWGSSTHYYYGMDV

SEQ ID NO: 121 - protein, 10 aa, synthetic construct
  REGION 1..10: note = Description of Artificial Sequence: Synthetic peptide
SSNIGSNYVY

SEQ ID NO: 122 - protein, 11 aa, synthetic construct
  REGION 1..11: note = Description of Artificial Sequence: Synthetic peptide
LLIYRNNQRPS

SEQ ID NO: 123 - protein, 10 aa, synthetic construct
  REGION 1..10: note = Description of Artificial Sequence: Synthetic peptide
AAWDDSLSGV

SEQ ID NO: 124 - protein, 9 aa, synthetic construct
  REGION 1..9: note = Description of Artificial Sequence: Synthetic peptide
YTFTGYYMH

SEQ ID NO: 125 - protein, 15 aa, synthetic construct
  REGION 1..15: note = Description of Artificial Sequence: Synthetic peptide
WMGWINPNGGGTKYA

SEQ ID NO: 126 - protein, 10 aa, synthetic construct
  REGION 1..10: note = Description of Artificial Sequence: Synthetic peptide
TLSDYSSGGP

SEQ ID NO: 127 - protein, 10 aa, synthetic construct
  REGION 1..10: note = Description of Artificial Sequence: Synthetic peptide
SSNIGSNYVY

SEQ ID NO: 128 - protein, 11 aa, synthetic construct
  REGION 1..11: note = Description of Artificial Sequence: Synthetic peptide
LLIYRNNQRPS

SEQ ID NO: 129 - protein, 10 aa, synthetic construct
  REGION 1..10: note = Description of Artificial Sequence: Synthetic peptide
AAWDDSLSGV

SEQ ID NO: 130 - protein, 9 aa, synthetic construct
  REGION 1..9: note = Description of Artificial Sequence: Synthetic peptide
YTFTGYHVH

SEQ ID NO: 131 - protein, 15 aa, synthetic construct
  REGION 1..15: note = Description of Artificial Sequence: Synthetic peptide
WMGWINPDSGGTNFA

SEQ ID NO: 132 - protein, 6 aa, synthetic construct
  REGION 1..6: note = Description of Artificial Sequence: Synthetic peptide
RRSLDY

SEQ ID NO: 133 - protein, 10 aa, synthetic construct
  REGION 1..10: note = Description of Artificial Sequence: Synthetic peptide
SSNIGSNYVY

SEQ ID NO: 134 - protein, 11 aa, synthetic construct
  REGION 1..11: note = Description of Artificial Sequence: Synthetic peptide
LLIYRNNQRPS

SEQ ID NO: 135 - protein, 10 aa, synthetic construct
  REGION 1..10: note = Description of Artificial Sequence: Synthetic peptide
AAWDDSLNGV

SEQ ID NO: 136 - protein, 9 aa, synthetic construct
  REGION 1..9: note = Description of Artificial Sequence: Synthetic peptide
FTFSNAWMS

SEQ ID NO: 137 - protein, 16 aa, synthetic construct
  REGION 1..16: note = Description of Artificial Sequence: Synthetic peptide
WVGRIKSKTDGGTTDY

SEQ ID NO: 138 - protein, 6 aa, synthetic construct
  REGION 1..6: note = Description of Artificial Sequence: Synthetic peptide
ASLVDY

SEQ ID NO: 139 - protein, 10 aa, synthetic construct
  REGION 1..10: note = Description of Artificial Sequence: Synthetic peptide
SSNIGSNYVY

SEQ ID NO: 140 - protein, 11 aa, synthetic construct
  REGION 1..11: note = Description of Artificial Sequence: Synthetic peptide
LLIYRNNQRPS

SEQ ID NO: 141 - protein, 10 aa, synthetic construct
  REGION 1..10: note = Description of Artificial Sequence: Synthetic peptide
AAWDDSLSGP

SEQ ID NO: 142 - protein, 9 aa, synthetic construct
  REGION 1..9: note = Description of Artificial Sequence: Synthetic peptide
YTFTKYGIS

SEQ ID NO: 143 - protein, 14 aa, synthetic construct
  REGION 1..14: note = Description of Artificial Sequence: Synthetic peptide
WMGWISAYNVDTKY

SEQ ID NO: 144 - protein, 6 aa, synthetic construct
  REGION 1..6: note = Description of Artificial Sequence: Synthetic peptide
RRGLDY

SEQ ID NO: 145 - DNA, 905 bp, synthetic construct
  misc_feature 1..905: note = Description of Artificial Sequence: Synthetic polynucleotide
  modified_base 8: mod_base = OTHER; note = a, c, t, g, unknown or other
  modified_base 12: mod_base = OTHER; note = a, c, t, g, unknown or other
  modified_base 14: mod_base = OTHER; note = a, c, t, g, unknown or other
  modified_base 738: mod_base = OTHER; note = a, c, t, g, unknown or other
  modified_base 849: mod_base = OTHER; note = a, c, t, g, unknown or other
  source 1..905: mol_type = other DNA
cagctgantacngncgacgatgacaagctttcctatgagctgacacagccaccctcaatgtccgtgtccccaggacagacagccagcatcacctgctctggagataaattgggagataaatatgcttcctggtatcagcagaagccaggccagtcccctgtgctggtcatctatcaagatagcaagcggccctcagggatccctgagcgattctctggctccaactctgggaacacagccactctgaccatcagcgggacccaggctatggatgaggctgactattactgtcaggcgtgggacagcagcactgcggtattcggtggagggaccaagctcaccgtcctaggtgagggtaaatcttccggatctggttccgaatccaaagctagccaggtgcagctgcaggagtcgggcccaggactggtgaagccttcacagaccctgtccctcacctgcactgtctctggtggctccatcagcagtgatgattactactggagttggatccgccagaccccagggaagggcctggagtggattgggtacatctattacagtgggatcacctactacaacccgtccctcaagagtcgagttaccatatcagtagacacgtcgaagaaccagttctccctgaagctgagctctgtgactgccgcagacacggccgtgtattactgtgccagagaggggtgtaatgatggtgtatgctataatggggtctttgactactgnggccagggcaccctggtcaccgtctcctcagtcgacccattcgtttctgaatatcaaggccaatcgtctgacctgcctcaacctcctgtcaatgctggcggcggctctganggaggcggttccggtggtggctctggttccggtgattttgattatgaaaagatggc

SEQ ID NO: 146 - protein, 246 aa, synthetic construct
  REGION 1..246: note = Description of Artificial Sequence: Synthetic polypeptide
SYELTQPPSMSVSPGQTASITCSGDKLGDKYASWYQQKPGQSPVLVIYQDSKRPSGIPERFSGSNSGNTATLTISGTQAMDEADYYCQAWDSSTAVFGGGTKLTVLGEGKSSGSGSESKASQVQLQESGPGLVKPSQTLSLTCTVSGGSISSDDYYWSWIRQTPGKGLEWIGYIYYSGITYYNPSLKSRVTISVDTSKNQFSLKLSSVTAADTAVYYCAREGCNDGVCYNGVFDYWGQGTLVTVSS

SEQ ID NO: 147 - DNA, 729 bp, synthetic construct
  misc_feature 1..729: note = Description of Artificial Sequence: Synthetic polynucleotide
  source 1..729: mol_type = other DNA
cagtctgccctgactcagcctgcctccgtgtctgggtctcctggacagtcgatcaccatctcctgcgctggaaccagcagtgacgttggtacttataactatgtctcctggtaccaacaacacccaggcaaagcccccaaactcatgatttatgatgtcagtaagcggccctcaggggtccctgatcgcttctctggctccaagtctggcaacacggcctccctgaccatctctgggctccaggctgaggacgaggctgattattactgctactcatatacaaccagcagcacttgggtgttcggcggagggaccaaggtcaccgtcctaggagagggtaaatcttccggatctggttccgaaagcaaggctagccaggtgcagctgcaggagtcgggcccaggactgctgaagccttcgcagaccctgtccctcacctgcactgtctccggtgactccatcggcagtggtgattactactggagttggatccgccagcccccagggaagggcctggaatggattgggtacagctatcacactgggagcaccgactacaacccgtccctcaagagtcgagtttccatatcagtggacaggtccaagaaccagttctcccttaaactgaggtctgtgactgccgcagacacggccgtgtattactgtgccagagattattatggatatttgggttactggggccagggaaccctggtcaccgtctcctca

SEQ ID NO: 148 - protein, 243 aa, synthetic construct
  REGION 1..243: note = Description of Artificial Sequence: Synthetic polypeptide
QSALTQPASVSGSPGQSITISCAGTSSDVGTYNYVSWYQQHPGKAPKLMIYDVSKRPSGVPDRFSGSKSGNTASLTISGLQAEDEADYYCYSYTTSSTWVFGGGTKVTVLGEGKSSGSGSESKASQVQLQESGPGLLKPSQTLSLTCTVSGDSIGSGDYYWSWIRQPPGKGLEWIGYSYHTGSTDYNPSLKSRVSISVDRSKNQFSLKLRSVTAADTAVYYCARDYYGYLGYWGQGTLVTVSS

SEQ ID NO: 149 - DNA, 738 bp, synthetic construct
  misc_feature 1..738: note = Description of Artificial Sequence: Synthetic polynucleotide
  source 1..738: mol_type = other DNA
gacatccagatgacccagtctccatcctccctgtctgcatctgtaggagacagagtcaccatcacttgccgggcaagtcagagcattagcagctatttaaattggtatcagcagaaaccagggaaagcccctaagctcctgatctatgctgcatccagtttgcaaagtggggtcccatcaaggttcagtggcagtggatctgggacagatttcactctcaccatcagcagtctgcaacctgaagattttgcaacttactactgtcaacagagttacagtacccctcgaacgttcggccaagggaccaaagtggatatcaaagagggtaaatcttccggatctggttccgaatccaaagctagccaggtgcagctgcaggagtcgggcccaggactggtgaagccttcacagaccctgtccctcacctgcactgtctctggtggctccatcagcagtgatgattactactggagttggatccgccagaccccagggaagggcctggagtggattgggtacatctattacagtgggatcacctactacaacccgtccctcaagagtcgagttaccatatcagtagacacgtcgaagaaccagttctccctgaagctgagctctgtgactgccgcagacacggccgtgtattactgtgccagagaggggtgtaatgatggtgtatgctataatggggtctttgactactggggccagggcaccctggtcaccgtctcctca

SEQ ID NO: 150 - protein, 246 aa, synthetic construct
  REGION 1..246: note = Description of Artificial Sequence: Synthetic polypeptide
DIQMTQSPSSLSASVGDRVTITCRASQSISSYLNWYQQKPGKAPKLLIYAASSLQSGVPSRFSGSGSGTDFTLTISSLQPEDFATYYCQQSYSTPRTFGQGTKVDIKEGKSSGSGSESKASQVQLQESGPGLVKPSQTLSLTCTVSGGSISSDDYYWSWIRQTPGKGLEWIGYIYYSGITYYNPSLKSRVTISVDTSKNQFSLKLSSVTAADTAVYYCAREGCNDGVCYNGVFDYWGQGTLVTVSS

SEQ ID NO: 151 - DNA, 738 bp, synthetic construct
  misc_feature 1..738: note = Description of Artificial Sequence: Synthetic polynucleotide
  source 1..738: mol_type = other DNA
ctgcctgtgctgactcagccaccctcagcgtcggggacccccgggcagagggtcaccatctcttgttctggaagcagctccaacatcggaggtaatactgtaaactggtatcaccaactcccaggatcggcccccaaactcctcatctatggtgatgatctgcggccctcaggggtccctgaccgattctccggctccaagtctggcacgtcagcctccctggccatcagtaggttccagtctggggatgaggctgattattactgtgcagcatgggatgacagcctgaatgcttatgtcttcggaactgggaccaagctcaccgtcctaggtgagggtaaatcttccggatctggttccgactccaaagctagcgaggtgcagctggtggggtctgggggaggcgtggtccagcctgggaggtccctgagactctcctgtgcagcctctggattcaccttcagtaactatgctatgcactgggtccgccaggctccaggcaaggggctggagtgggtggcagttatatcatatgatggaagtaataaatactacgcagactccgtgaagggccgattcaccatctccagagacaattccaagaacacgctgtatctgcaaatgaacagcctgagagctgaggacacggctgtgtattactgtgcgagagtccgctactatggttcggggagtcccattgggtactggggccagggaaccctggtcaccgtctcctca

SEQ ID NO: 152 - protein, 246 aa, synthetic construct
  REGION 1..246: note = Description of Artificial Sequence: Synthetic polypeptide
LPVLTQPPSASGTPGQRVTISCSGSSSNIGGNTVNWYHQLPGSAPKLLIYGDDLRPSGVPDRFSGSKSGTSASLAISRFQSGDEADYYCAAWDDSLNAYVFGTGTKLTVLGEGKSSGSGSDSKASEVQLVGSGGGVVQPGRSLRLSCAASGFTFSNYAMHWVRQAPGKGLEWVAVISYDGSNKYYADSVKGRFTISRDNSKNTLYLQMNSLRAEDTAVYYCARVRYYGSGSPIGYWGQGTLVTVSS

SEQ ID NO: 153 - DNA, 729 bp, synthetic construct
  misc_feature 1..729: note = Description of Artificial Sequence: Synthetic polynucleotide
  source 1..729: mol_type = other DNA
cagtctgccctgactcagcctgcctccgtgtctgggtctcctggacagtcgatcaccatctcctgcactggaaccagcagtgacgttggtggttataagtctgtctcctggtaccaacaacacccaggcaaagcccccaaactcatgatttatgatgtcagtaatcggccctcaggggtttctgatcgcttctctggctccaagtctggcaacacggcctccctgaccatctctgggctccaggctgaggacgaggctgattattactgcagctcttacacaagcagcagctccctttgggtgttcggcggagggaccaagctcaccgtcctaggagagggtaaatcttccggatctggttccgaaagcaaggctagccaggttcagctggtgcagtctggggctgaggtgaagaagcctgggtcctcggtgaaggtctcctgcaaggcttctggaggcaccttcagcagctatgctatcagctgggtgcgacaggcccctggacaagggcttgagtggatgggaaggatcatccctatccttggtatagcaaactacgcacagaagttccagggcagagtcaccatgaccgaggacacatctacagacacagcctacatggagctgagcagcctgagatctgaggacacggccgtgtattactgtgcaacagatctgtggggagtgggagcagattggggccagggaaccctggtcaccgtctcctca

SEQ ID NO: 154 - protein, 243 aa, synthetic construct
  REGION 1..243: note = Description of Artificial Sequence: Synthetic polypeptide
QSALTQPASVSGSPGQSITISCTGTSSDVGGYKSVSWYQQHPGKAPKLMIYDVSNRPSGVSDRFSGSKSGNTASLTISGLQAEDEADYYCSSYTSSSSLWVFGGGTKLTVLGEGKSSGSGSESKASQVQLVQSGAEVKKPGSSVKVSCKASGGTFSSYAISWVRQAPGQGLEWMGRIIPILGIANYAQKFQGRVTMTEDTSTDTAYMELSSLRSEDTAVYYCATDLWGVGADWGQGTLVTVSS

SEQ ID NO: 155 - DNA, 738 bp, synthetic construct
  misc_feature 1..738: note = Description of Artificial Sequence: Synthetic polynucleotide
  source 1..738: mol_type = other DNA
ctgcctgtgctgactcagcctgcctccgtgtctgggtctcctggacagtcgatcaccttctcctgcactggaaccaacactgacattggttattataattatgtctcctggtaccaacaactcccaggcaaagcccccaaactcttgatttttgaggtcgataatcggccctcaggggtccctagtcgcttctctggctccaagtctggcaacacggcctccctgaccatctctgggctccaggctgaggacgaggctgattattactgcagctcatattcaacctataatattttgctcttcggcggagggaccaagctcaccgtcctaggtgagggtaaatcttccggatctggttccgaatccaaagctagcgaggtgcagctgttggagtctgaggctgaggtgaagaagcctggggcctcagtgaaggtctcctgcaaggcttctggatacaccttcaccggctactatatgcactgggtgcgacaggcccctggacaagggcttgagtggatgggacggatcaaccctaacagtggtggcacaaactatgcacagaagtttcagggcagggtcaccatgaccagggacacgtccatcagcacagcctacatggagctgagcaggctgagatctgacgacacggccgtgtattactgtgcgagagaccccacgtattacgatattttgactggtccggagtactggggccagggaaccgtcaccgtctcctca

SEQ ID NO: 156 - protein, 246 aa, synthetic construct
  REGION 1..246: note = Description of Artificial Sequence: Synthetic polypeptide
LPVLTQPASVSGSPGQSITFSCTGTNTDIGYYNYVSWYQQLPGKAPKLLIFEVDNRPSGVPSRFSGSKSGNTASLTISGLQAEDEADYYCSSYSTYNILLFGGGTKLTVLGEGKSSGSGSESKASEVQLLESEAEVKKPGASVKVSCKASGYTFTGYYMHWVRQAPGQGLEWMGRINPNSGGTNYAQKFQGRVTMTRDTSISTAYMELSRLRSDDTAVYYCARDPTYYDILTGPEYWGQGTVTVSS

SEQ ID NO: 157 - DNA, 702 bp, synthetic construct
  misc_feature 1..702: note = Description of Artificial Sequence: Synthetic polynucleotide
  source 1..702: mol_type = other DNA
gaaatagtgatgacacagtctccagccaccctgtctgtgtctccaggggaaagagccaccctctcctgcagggccagtcagagtgttagcagcaacttagcctggtaccagcagaaacctggccaggctcccaggctcctcatctatggtgcatccagcagggccactggcatcccagacaggttcagtggcagtgggtctgggacagacttcactctcaccatcagcagactggagcctgaggattttgcagtgtattactgtcagcaatatatttactcaccgtacacttttggccaggggaccaaagtggatatcaaagagggtaaatcttccggatctggttccgaatccaaagctagcgaggtgcagctggtgcagtctggggctgaggtgaagaagcctggggcctcagtgaaggtctcctgcaaggcctctggatacaacttcgccggctactatgttcactgggtgcgacaggcccctggacaagggcttgagtggatgggatggatcaaccctaacagtggtggcacagactatgcacagaagtttcagggcagggtcaccatgaccagggacacgtccatcagcacagcctacatggacctgagtaggctgagatctgacgacacggccgtctattactgtgcgaggaatctacagttttttcggccagggaccctggtcaccgtctcctca

SEQ ID NO: 158 - protein, 234 aa, synthetic construct
  REGION 1..234: note = Description of Artificial Sequence: Synthetic polypeptide
EIVMTQSPATLSVSPGERATLSCRASQSVSSNLAWYQQKPGQAPRLLIYGASSRATGIPDRFSGSGSGTDFTLTISRLEPEDFAVYYCQQYIYSPYTFGQGTKVDIKEGKSSGSGSESKASEVQLVQSGAEVKKPGASVKVSCKASGYNFAGYYVHWVRQAPGQGLEWMGWINPNSGGTDYAQKFQGRVTMTRDTSISTAYMDLSRLRSDDTAVYYCARNLQFFRPGTLVTVSS

SEQ ID NO: 159 - DNA, 720 bp, synthetic construct
  misc_feature 1..720: note = Description of Artificial Sequence: Synthetic polynucleotide
  source 1..720: mol_type = other DNA
tcctatgagctgactcagccactctcagtgtcagtggccctgggacagacggccaggattacctgtgggggaaacaacattggaagtaaaaatgtgcactggtaccagcagaagccaggccaggcccctgtgctggtcatctatgatgatagcgaccggccctcagggacctccgagcgattctctggctccaactctgggaacacagccactctgaccatcagcgggacccaggctatggatgaggctgactattactgtcaggcgtgggacagcagcactgcagtggtattcggcggagggaccaagctcaccgtcctaggtgagggtaaatcttccggatctggttccgaatccaaagctagccaggtgcagctgcaggagtcgggcccaggactggtgaagccttcggagaccctgtccctcacctgcactgtctctggtggctccatcagcagtagtagttactactggggctggatccgccagcccccagggaaggggctggagtggattgggagtatctattatagtgggagcacctactacaacccgtccctcaagagtcgagccaccatatccgtagacacgtccaagaaccagttctccctgaagatgacctcagtgaccgccgcagacacggccatatattactgtgcgagacaggtgggccctgtgttaaagtcggtatctcagggcaccctggtcaccgtcacctca

SEQ ID NO: 160 - protein, 240 aa, synthetic construct
  REGION 1..240: note = Description of Artificial Sequence: Synthetic polypeptide
SYELTQPLSVSVALGQTARITCGGNNIGSKNVHWYQQKPGQAPVLVIYDDSDRPSGTSERFSGSNSGNTATLTISGTQAMDEADYYCQAWDSSTAVVFGGGTKLTVLGEGKSSGSGSESKASQVQLQESGPGLVKPSETLSLTCTVSGGSISSSSYYWGWIRQPPGKGLEWIGSIYYSGSTYYNPSLKSRATISVDTSKNQFSLKMTSVTAADTAIYYCARQVGPVLKSVSQGTLVTVTS

SEQ ID NO: 161 - DNA, 717 bp, synthetic construct
  misc_feature 1..717: note = Description of Artificial Sequence: Synthetic polynucleotide
  source 1..717: mol_type = other DNA
gaagtgcagctgctggaaagcggcggtggtctggttcagccgggtggcagcctgcgtctgagctgtgcggcgagcggctttacctttagcagctatgccatgagctgggtgcgtcaggcaccgggcaaaggcctggaatgggtgagcgcgattagcggcagcggcggcagcacctattatgcggatagcgtgaaaggccgttttaccattagccgtgataacagcaaaaacaccctgtatctgcagatgaacagcctgcgtgcggaagataccgcggtgtattattgcgcgaaaagcgccagcttctttgattattggggccagggcaccctggttaccgttagcagcggtggaggcggttctggtggaggcggttcgggtgacggaagttcagaaattgtgctgacccagagcccgggcacgctgtctctgagcccgggtgaacgtgcgaccctgagctgtcgtgcgagccagagcgtgagcagcagctatctggcctggtatcagcagaaaccgggccaggcaccgcgtctgctgatttatggcgcgagcagccgtgcgaccggcattccggatcgttttagcggcagcggtagcggcaccgattttaccctgaccattagccgtctggaaccggaagattttgcggtgtattattgccagcagcatttccgttggccgtggacctttggccagggcaccaaagtggaaattaaa

SEQ ID NO: 162 - protein, 239 aa, synthetic construct
  REGION 1..239: note = Description of Artificial Sequence: Synthetic polypeptide
EVQLLESGGGLVQPGGSLRLSCAASGFTFSSYAMSWVRQAPGKGLEWVSAISGSGGSTYYADSVKGRFTISRDNSKNTLYLQMNSLRAEDTAVYYCAKSASFFDYWGQGTLVTVSSGGGGSGGGGSGDGSSEIVLTQSPGTLSLSPGERATLSCRASQSVSSSYLAWYQQKPGQAPRLLIYGASSRATGIPDRFSGSGSGTDFTLTISRLEPEDFAVYYCQQHFRWPWTFGQGTKVEIK

SEQ ID NO: 163 - DNA, 726 bp, synthetic construct
  misc_feature 1..726: note = Description of Artificial Sequence: Synthetic polynucleotide
  source 1..726: mol_type = other DNA
tcctatgagctgactcagccaccctcagcgtctgggacccccgggcagaaggtcaccatctcttgttctggaagcagctccaacatcggaagtaatactgtaaactggtaccagcagctcccaggaacggcccccaaactcctcatctatagtaataatcagcggccctcaggggtccctgaccgattctctggctccaagtctggcacctcagcctccctggccatcagtgggctccagtctgaggatgaggctgattattactgtgcagcgtgggatgacagcctgaatggtgtggttttcggcggagggaccaaggtgaccgtcctaggtgagggtaaatcttccggatctggttccgaatccaaagctagccaggtgcagctgcaggagtcgggcccaggactggtgaagccttcacagaccctgtccctcacctgcactgtctctggtgcctccatcagcagtggtggttactactggagctggatccgccagcacccagggaagggcctggagtggattgggtacagctattacagtgggagcacctactacaacccgtccctcaagagtcgagttaccatatcagtagacacgtccaagaaccagttctccctgtacctgacctctgtgaccgctgcggacacggccgtatatcattgtgcgagagggggggtcaggtttgacctctggggccagggcaccctggtcaccgtctcctca

SEQ ID NO: 164 - protein, 242 aa, synthetic construct
  REGION 1..242: note = Description of Artificial Sequence: Synthetic polypeptide
SYELTQPPSASGTPGQKVTISCSGSSSNIGSNTVNWYQQLPGTAPKLLIYSNNQRPSGVPDRFSGSKSGTSASLAISGLQSEDEADYYCAAWDDSLNGVVFGGGTKVTVLGEGKSSGSGSESKASQVQLQESGPGLVKPSQTLSLTCTVSGASISSGGYYWSWIRQHPGKGLEWIGYSYYSGSTYYNPSLKSRVTISVDTSKNQFSLYLTSVTAADTAVYHCARGGVRFDLWGQGTLVTVSS

SEQ ID NO: 165 - DNA, 762 bp, synthetic construct
  misc_feature 1..762: note = Description of Artificial Sequence: Synthetic polynucleotide
  source 1..762: mol_type = other DNA
tcctatgagctgactcagccaccctcggtgtcagtgtccccaggacaaacggccaggatcacctgctctggagatgcattgccaaaaaaatatgcttattggtaccagcagaagtcaggccaggcccctgtgctggtcatctatgaggacagcaaacgaccctccgggatccctgagagattctctggctccagctcagggacaatggccaccttgactgtcagtggggcccaggtggaggatgaagctgactactactgttactcaacagacagcagtggtaatccagtgttcggcggagggaccaagctgaccgtcctaggtgagggtaaatcttccggatctggttccgaatccaaagctagcgaggtgcagctgttggagtctgggggaggcttggtacagcctggggggtccctgagactctcctgtgcagcctctggattcacctttagcagctatgccatgagctgggtccgccaggctccagggaaggggctggagtgggtctcagctattagtggtagtggtggtagcacatactacgcagactccgtgaagggccggttcaccatctccagagacaattccaagaacacgctgtatctgcaaatgaacagcctgagagccgaggacacggccgtatattactgtgcgaaaattccttggggtgattacgatttttggagtggttattataccaggcccggtcactccggtatggacgtctggggccaaggcaccctggtcaccgtctcctca

SEQ ID NO: 166 - protein, 254 aa, synthetic construct
  REGION 1..254: note = Description of Artificial Sequence: Synthetic polypeptide
SYELTQPPSVSVSPGQTARITCSGDALPKKYAYWYQQKSGQAPVLVIYEDSKRPSGIPERFSGSSSGTMATLTVSGAQVEDEADYYCYSTDSSGNPVFGGGTKLTVLGEGKSSGSGSESKASEVQLLESGGGLVQPGGSLRLSCAASGFTFSSYAMSWVRQAPGKGLEWVSAISGSGGSTYYADSVKGRFTISRDNSKNTLYLQMNSLRAEDTAVYYCAKIPWGDYDFWSGYYTRPGHSGMDVWGQGTLVTVSS

SEQ ID NO: 167 - DNA, 726 bp, synthetic construct
  misc_feature 1..726: note = Description of Artificial Sequence: Synthetic polynucleotide
  source 1..726: mol_type = other DNA
caggctgtgctgactcagccgccctcagtgtctggggccccagggcagagggtcaccatctcctgcgctgggagcagctccaacatcggggcaggttatgatgtacactggtaccaacagcttccaggaacagcccccaagctcctcatctttgatagctccaatcggccctcaggggtccctgaccgattctctggctccaagtccggcacctcagcctccctggccatcactgggctccaggctgaggatgaggctgattattactgccagtcctatgacttcaggctgagtggttctatggtcttcggcggagggaccaagctgaccgtcctaggtgagggtaaatcttccggatctggttccgaatccaaagctagcgaggtgcagctggtggagtctgggggaggcctggtcaagcctggggggtccctgagactctcctgtgcagcctctggattcaccttcagggcctatcccatgagctgggtccgccaggctccagggaaggggctggaatgggtctcatccattacttctagtggcagttactacgcagactcagtgaagggtcgatttaccatctccagagacaacgccaagagttcactgtatctccaaatgaacagcctgagagccgacgacacggctgtctattactgtgcgagagtgggagttactgactttgactactggggccagggaaccctggtcaccgtctcctca

SEQ ID NO: 168 - protein, 242 aa, synthetic construct
  REGION 1..242: note = Description of Artificial Sequence: Synthetic polypeptide
QAVLTQPPSVSGAPGQRVTISCAGSSSNIGAGYDVHWYQQLPGTAPKLLIFDSSNRPSGVPDRFSGSKSGTSASLAITGLQAEDEADYYCQSYDFRLSGSMVFGGGTKLTVLGEGKSSGSGSESKASEVQLVESGGGLVKPGGSLRLSCAASGFTFRAYPMSWVRQAPGKGLEWVSSITSSGSYYADSVKGRFTISRDNAKSSLYLQMNSLRADDTAVYYCARVGVTDFDYWGQGTLVTVSS

SEQ ID NO: 169 - DNA, 735 bp, synthetic construct
  misc_feature 1..735: note = Description of Artificial Sequence: Synthetic polynucleotide
  source 1..735: mol_type = other DNA
cagtctgtgctgactcagccgccctcagcgtctgggacccccgggcagagggtcaccatctcttgttctggaagcagctccaacatcggaactaattatgtatactggtaccagcagctcccaggaacggcccccaaactcctcatctataggaataatcagcggccctcaggggcccctgaccgattctctggctccaagtctggcacctcagcctccctggccatcagtgggctccggtccgaggatgaggctgattattactgtgcagcatgggatgacagcctgagtggttgggtgttcggcggagggaccaaggtgaccgtcctaggtgagggtaaatcttccggatctggttccgaatccaaagctagcgaggtgcagctgttggagtctgggggaggcttggtacagcctggggggtccctgagactctcctgtgcagcctctggattcacctttagcagctatgccatgagctgggtccgccaggctccagggaaggggctggagtgggtctcagctattagtggtagtggtggtagcacatactacgcagactccgtgaagggccggttcaccatctccagagacaattccaagaacacgctgtatctgcaaatgaacagcctgagagccgaggacacggccgtatattactgtgcgaaaagtatcagaactgggagcgggtactttgactactggggccagggcaccctggtcaccgtctcctca

SEQ ID NO: 170 - protein, 245 aa, synthetic construct
  REGION 1..245: note = Description of Artificial Sequence: Synthetic polypeptide
QSVLTQPPSASGTPGQRVTISCSGSSSNIGTNYVYWYQQLPGTAPKLLIYRNNQRPSGAPDRFSGSKSGTSASLAISGLRSEDEADYYCAAWDDSLSGWVFGGGTKVTVLGEGKSSGSGSESKASEVQLLESGGGLVQPGGSLRLSCAASGFTFSSYAMSWVRQAPGKGLEWVSAISGSGGSTYYADSVKGRFTISRDNSKNTLYLQMNSLRAEDTAVYYCAKSIRTGSGYFDYWGQGTLVTVSS

SEQ ID NO: 171 - DNA, 738 bp, synthetic construct
  misc_feature 1..738: note = Description of Artificial Sequence: Synthetic polynucleotide
  source 1..738: mol_type = other DNA
cagtctgtgctgacgcagccgccctcagcgtctgggacccccgggcagagggtcaccatctcttgttctggaagcagctccaacatcggaagtaattatgtatactggtaccagcagctcccaggaacggcccccaaactcctcatctataggaataatcagcggccctcaggggtccctgaccgattctctggctccaagtctggcacctcagcctccctggccatcagtgggctccggtccgaggatgaggctgattattactgtgcagcatgggatgacagcctgagtggttgggtgttcggcggagggaccaagctcaccgtcctaggtgagggtaaatcttccggatctggttccgaatccaaagctagccaggttcagctgcagtctggggctgaggtgaagaagcctggggcctcagtgaaggtttcctgcaaggcatctggatacaccttcaccagctactatatgcactgggtgcgacaggcccctggacaagggcttgagtggatgggaataatcaaccctagtggtggtagcacaagctacgcacagaagttccagggcagagtcaccatgaccagggacacgtccacgagcacagtctacatggagctgagcagcctgagatctgaggacacggccgtgtattactgtgcgagagatctcctcctctatggtcgcgggggcggtttccagcactggggccagggaaccctggtcaccgtctcctca

SEQ ID NO: 172 - protein, 246 aa, synthetic construct
  REGION 1..246: note = Description of Artificial Sequence: Synthetic polypeptide
QSVLTQPPSASGTPGQRVTISCSGSSSNIGSNYVYWYQQLPGTAPKLLIYRNNQRPSGVPDRFSGSKSGTSASLAISGLRSEDEADYYCAAWDDSLSGWVFGGGTKLTVLGEGKSSGSGSESKASQVQLQSGAEVKKPGASVKVSCKASGYTFTSYYMHWVRQAPGQGLEWMGIINPSGGSTSYAQKFQGRVTMTRDTSTSTVYMELSSLRSEDTAVYYCARDLLLYGRGGGFQHWGQGTLVTVSS

SEQ ID NO: 173 - DNA, 717 bp, synthetic construct
  misc_feature 1..717: note = Description of Artificial Sequence: Synthetic polynucleotide
  modified_base 587: mod_base = OTHER; note = a, c, t, g, unknown or other
  source 1..717: mol_type = other DNA
tcttctgagctgactcaggaccctgctgtgtctgtggccttaggacagacagtcaggatcacatgccaaggagacagcctcagaagctattatgcaagctggtaccagcagaagccaggacaggcccctgtacttgtcatctatggtaaaaacaaccggccctcagggatcccagcccgattctctggctccagctcaggaaacacagcttccttgaccatcactggggctcaggcggaagatgaggctgactattactgtaactcccgggacaacagtggtaagcatctttgggtgttcggcggagggaccaagctcaccgtcctaggtgagggtaaatcttccggatctggttccgaatccaaagctagcgaggtgcagctggtgcagtctgggggaggtgtggtacggcctggggggtccctgagactctcctgtgcagcctctggattcacctttgatgattatggcatgagctgggtccgccaagctccagggaaggggctggagtgggtctctggtattaattggaatggtggtagcacaggttatgcagactctgtgaagggccgattcaccatctccanagacaacgccaagaactccctgtatctgcaaatgaacagtctgagagccgaggacacggccttgtattactgtgcgaggaaatctacaggtgactactggggccagggaaccctggtcaccgtctcttca

SEQ ID NO: 174 - protein, 239 aa, synthetic construct
  REGION 1..239: note = Description of Artificial Sequence: Synthetic polypeptide
SSELTQDPAVSVALGQTVRITCQGDSLRSYYASWYQQKPGQAPVLVIYGKNNRPSGIPARFSGSSSGNTASLTITGAQAEDEADYYCNSRDNSGKHLWVFGGGTKLTVLGEGKSSGSGSESKASEVQLVQSGGGVVRPGGSLRLSCAASGFTFDDYGMSWVRQAPGKGLEWVSGINWNGGSTGYADSVKGRFTISTDNAKNSLYLQMNSLRAEDTALYYCARKSTGDYWGQGTLVTVSS

SEQ ID NO: 175 - DNA, 738 bp, synthetic construct
  misc_feature 1..738: note = Description of Artificial Sequence: Synthetic polynucleotide
  source 1..738: mol_type = other DNA
cagtctgtgctgacgcagccgccctcagtgtctggggccccagggcagagggtcaccatctcctgcactgggagcagctccaacatcggggcaggttatgatgtacactggtaccagcagcttccaggaacagcccccaaactcctcatctatggtaacagcaatcggccctcaggggtccctgaccgattctctggctccaagtctggcacctcagcctccctggccatcagtgggctccagtctgaggatgaggctgattattactgtgcagcatgggatgacagcctgaatggtccgagaatggtattcggcggagggaccaagctgaccgtcctaggtgagggtaaatcttccggatctggttccgaatccaaagctagcgaggtgcagctggtgcagtctgggggaggcttggtcaagcctggagggtccctgagactctcctgtgcagcctctggattcaccttcagtgactactacatgagctggatccgccaggctccagggaaggggctggagtgggtttcatacattagtagtagtagtagttacacaaactacgcagactctgtgaagggccgattcaccatctccagagacaacgccaagaactcactgtatctgcaaatgaacagcctgagagccgaggacacggctgtgtattactgtgcgagagttaactactactacggtatggacgtctggggccaaggcaccctggtcaccgtctcttca

SEQ ID NO: 176 - protein, 246 aa, synthetic construct
  REGION 1..246: note = Description of Artificial Sequence: Synthetic polypeptide
QSVLTQPPSVSGAPGQRVTISCTGSSSNIGAGYDVHWYQQLPGTAPKLLIYGNSNRPSGVPDRFSGSKSGTSASLAISGLQSEDEADYYCAAWDDSLNGPRMVFGGGTKLTVLGEGKSSGSGSESKASEVQLVQSGGGLVKPGGSLRLSCAASGFTFSDYYMSWIRQAPGKGLEWVSYISSSSSYTNYADSVKGRFTISRDNAKNSLYLQMNSLRAEDTAVYYCARVNYYYGMDVWGQGTLVTVSS

SEQ ID NO: 177 - DNA, 726 bp, synthetic construct
  misc_feature 1..726: note = Description of Artificial Sequence: Synthetic polynucleotide
  source 1..726: mol_type = other DNA
tcttctgagctgactcaggaccctgctgtgtctgtggccttgggacagacagtcagaatcacatgccaaggagacagcctcagaaaatattatgcaagctggtaccagcagaaggcaggacaggcccctgtacttgtcatctatggtaaaaacaaacggccctcagggatcccagaccgattctctggctccagctcaggaaacacagcttccttgaccatcactggggctcaggcggaagatgaggctgactattactgtaactcctgggacagcagtggtaaccacgtggtattcggcggagggaccaagctcaccgtcctaggtgagggtaaatcttccggatctggttccgaatccaaagctagccaggtgcagctgcaggagtcgggcccaggactggtgaagccttcacagaccctgtccctcacctgcactgtctctggtggctccatcagcagtggtggttactactggagctggatccgccagcacccagggaagggcctggagtggattgggtacatctattacagtgggagcacctactacaacccgtccctcaagggtcgagttaccatatcagtagacacgtctaagaaccagttctccctgaagctgagctctgtgactgccgcggacacggccgtgtattactgtgcgagagaagaagtgggagactggttcgacccctggggccaaggcaccctggtcaccgtctcctca

SEQ ID NO: 178 - protein, 242 aa, synthetic construct
  REGION 1..242: note = Description of Artificial Sequence: Synthetic polypeptide
SSELTQDPAVSVALGQTVRITCQGDSLRKYYASWYQQKAGQAPVLVIYGKNKRPSGIPDRFSGSSSGNTASLTITGAQAEDEADYYCNSWDSSGNHVVFGGGTKLTVLGEGKSSGSGSESKASQVQLQESGPGLVKPSQTLSLTCTVSGGSISSGGYYWSWIRQHPGKGLEWIGYIYYSGSTYYNPSLKGRVTISVDTSKNQFSLKLSSVTAADTAVYYCAREEVGDWFDPWGQGTLVTVSS

SEQ ID NO: 179 - DNA, 726 bp, synthetic construct
  misc_feature 1..726: note = Description of Artificial Sequence: Synthetic polynucleotide
  source 1..726: mol_type = other DNA
tcttctgagctgactcaggaccctgctgtgtctgtggccttgggacagacagtcagaatcacatgccaaggagacagcctcagaaaatattatgcaagctggtaccagcagaaggcaggacaggcccctgtacttgtcatctatggtaaaagcaaacggccctcagggatcccagaccgattctctggctccagctcaggaaacacagcttccttgaccatcactggggctcaggcggaagatgaggctgactattactgtaactcctgggacagcagtggtaaccacgtggtattcggcggagggaccaagctcaccgtcctaggtgagggtaaatcttccggatctggttccgaatccaaagctagccaggtgcagctgcaggagtcgggcccaggactggtgaagccttcacagaccctgtccctcacctgcactgtctctggtggctccatcagcagtggtggttactactggagctggatccgccagcacccagggaagggcctggagtggattgggtacatctattacagtgggagcacctactacaacccgtccctcaagggtcgagttaccatatcagtagacacgtctaagaaccagttctccctgaagctgagctctgtgactgccgcggacacggccgtgtattactgtgcgagagaagaagtgggagactggttcgacccctggggccagggcaccctggtcaccgtctcctca

SEQ ID NO: 180 - protein, 242 aa, synthetic construct
  REGION 1..242: note = Description of Artificial Sequence: Synthetic polypeptide
SSELTQDPAVSVALGQTVRITCQGDSLRKYYASWYQQKAGQAPVLVIYGKSKRPSGIPDRFSGSSSGNTASLTITGAQAEDEADYYCNSWDSSGNHVVFGGGTKLTVLGEGKSSGSGSESKASQVQLQESGPGLVKPSQTLSLTCTVSGGSISSGGYYWSWIRQHPGKGLEWIGYIYYSGSTYYNPSLKGRVTISVDTSKNQFSLKLSSVTAADTAVYYCAREEVGDWFDPWGQGTLVTVSS

SEQ ID NO: 181 - DNA, 726 bp, synthetic construct
  misc_feature 1..726: note = Description of Artificial Sequence: Synthetic polynucleotide
  source 1..726: mol_type = other DNA
cagtctgtgctgactcagccgccctcagcgtctgggacccccgggcagagggtcaccatctcttgttctggaagcagctccaacatcggaagtaattacgtatactggtaccagcagctcccaggaacggcccccaaactcctcatctataggaataatcagcggccctcaggggtccctgaccgattctctggctccaagtctggcacctcagcctccctggccatcagtgggctccggtccgaggatgaggctgattattactgtgcagcatgggatgacagcctgagtggtgtggtattcggcggagggaccaagctgaccgtcctaggtgagggtaaatcctccggatctggttccgaatccaaagctagccaggttcagctgcagtctggggctgaggtgaagaagcctggggcctcagtgaaggtctcctgcaaggcttctggatacaccttcaccggctactacatgcactgggtgcgacaggcccctggacaagggcttgagtggatgggatggatcaaccctaacggtggtggcacaaagtatgcacagaagtttcagggcagggtcaccatgaccagggacacgtccatcagcacagcctacatggagctgagcagtctgagatctgacgacacggccgtgtattactgtgcgacgctttctgactatagcagtggcggaccctggggccagggcaccctggtcaccgtctcctca

SEQ ID NO: 182 - protein, 242 aa, synthetic construct
  REGION 1..242: note = Description of Artificial Sequence: Synthetic polypeptide
QSVLTQPPSASGTPGQRVTISCSGSSSNIGSNYVYWYQQLPGTAPKLLIYRNNQRPSGVPDRFSGSKSGTSASLAISGLRSEDEADYYCAAWDDSLSGVVFGGGTKLTVLGEGKSSGSGSESKASQVQLQSGAEVKKPGASVKVSCKASGYTFTGYYMHWVRQAPGQGLEWMGWINPNGGGTKYAQKFQGRVTMTRDTSISTAYMELSSLRSDDTAVYYCATLSDYSSGGPWGQGTLVTVSS

SEQ ID NO: 183 - DNA, 717 bp, synthetic construct
  misc_feature 1..717: note = Description of Artificial Sequence: Synthetic polynucleotide
  source 1..717: mol_type = other DNA
caggctgtgctgactcagccaccctcagcgtctgggacccccgggcagagggtcaccatctcttgttctggaagcagctccaacatcggaagtaattatgtatactggtaccagcagctcccaggaacggcccccaaactcctcatctataggaataatcagcggccctcaggggtccctgaccgattctctggctccaagtctggcacctcagcctccctggccatcagtgggctccggtccgaggatgaggctgattattactgtgcagcatgggatgacagcctgagtggtgtggtattcggcggagggaccaagctcaccgtcctaggtgagggtaaatcttccggatctggttccgaatccaaagctagcgaggtgcagctggtgcagtctgggactgaggtgaagaggcctggggcctcagtgaaggtctcctgcaaggcttctggatacaccttcaccggctaccatgtgcactgggtgcgacaggcccctggacaagggcttgagtggatggggtggatcaaccctgacagtggtggcacaaactttgcacagaagtttcagggcagggtcaccatgaccagggacacgtccatcagcacagcctacatggaacttaccagcctgagatctgacgacacggccatttattactgtgcgagacgttcacttgactactggggccagggcaccctggtcaccgtctcctca

SEQ ID NO: 184 - protein, 239 aa, synthetic construct
  REGION 1..239: note = Description of Artificial Sequence: Synthetic polypeptide
QAVLTQPPSASGTPGQRVTISCSGSSSNIGSNYVYWYQQLPGTAPKLLIYRNNQRPSGVPDRFSGSKSGTSASLAISGLRSEDEADYYCAAWDDSLSGVVFGGGTKLTVLGEGKSSGSGSESKASEVQLVQSGTEVKRPGASVKVSCKASGYTFTGYHVHWVRQAPGQGLEWMGWINPDSGGTNFAQKFQGRVTMTRDTSISTAYMELTSLRSDDTAIYYCARRSLDYWGQGTLVTVSS

SEQ ID NO: 185 - DNA, 720 bp, synthetic construct
  misc_feature 1..720: note = Description of Artificial Sequence: Synthetic polynucleotide
  source 1..720: mol_type = other DNA
tcctatgagctgacacagccaccctcagcgtctgggacccccgggcagagggtcaccatctcttgttctggaagcagctccaacatcggaagtaattatgtatactggtaccagcagctcccaggaacggcccccaaactcctcatctataggaataatcagcggccctcaggggtccctgaccgattctctgcctccaagtctggcacctcagcctccctggccatcagtgggctccagtctgcggatgaggctgattattactgtgcagcatgggatgacagcctgaatggtgtggtattcggcggagggaccaagctgaccgtcctaggtgagggtaaatcttccggatctggttccgaatccaaagctagcgaggtgcagctggtgcagtctgggggaggcttggtccagcctggggggtcccttagactctcctgtgcagcctctggattcactttcagtaacgcctggatgagctgggtccgccaggctccagggaaggggctggagtgggttggccgtattaaaagcaaaactgatggtgggacaacagactacgctgcacccgtgaaaggcagattcaccatctcaagagatgattcaaaaaacacgctgtatctgcaaatgaacagcctgaaaaccgaggacacagccgtgtattactgtgctagcctggttgactactggggccagggcaccctggtcaccgtctcctca

SEQ ID NO: 186 - protein, 240 aa, synthetic construct
  REGION 1..240: note = Description of Artificial Sequence: Synthetic polypeptide
SYELTQPPSASGTPGQRVTISCSGSSSNIGSNYVYWYQQLPGTAPKLLIYRNNQRPSGVPDRFSASKSGTSASLAISGLQSADEADYYCAAWDDSLNGVVFGGGTKLTVLGEGKSSGSGSESKASEVQLVQSGGGLVQPGGSLRLSCAASGFTFSNAWMSWVRQAPGKGLEWVGRIKSKTDGGTTDYAAPVKGRFTISRDDSKNTLYLQMNSLKTEDTAVYYCASLVDYWGQGTLVTVSS

SEQ ID NO: 187 - DNA, 717 bp, synthetic construct
  misc_feature 1..717: note = Description of Artificial Sequence: Synthetic polynucleotide
  source 1..717: mol_type = other DNA
cagtctgtgctgactcagccgccctcagcgtctgggacccccgggcagagggtcaccatctcttgttctggaagcagctccaacatcggaagtaattatgtatactggtaccagcagctcccaggaacggcccccaaactcctcatctataggaataatcagcggccctcaggggtccctgaccgattctctggctccaagtctggcacctcagcctccctggccatcagtgggctccggtccgaggatgaggctgattattactgtgcagcatgggatgacagcctgagtggtccggtgttcggcggagggaccaaggtgaccgtcctaggtgagggtaaatcttccggatctggttccgaatccaaagctagcgaggtgcagctggtgcagtctggggctgttgtgaagaagcctggggcctcagtgaaggtctcctgcaaggcttctggctacacctttaccaagtatggtatcagctgggtgcgacaggcccctgaacaagggcttgagtggatgggatggatcagcgcttacaatgttgacacaaagtatgcacagaagttccagggcagagtcaccatgaccacagacacatccacgagcacagcctacatggaactgaggagccttagatctgacgacacggccgtgtattactgtgcgagaagagggcttgactactggggccagggcaccctggtcaccgtctcctca

SEQ ID NO: 188 - protein, 239 aa, synthetic construct
  REGION 1..239: note = Description of Artificial Sequence: Synthetic polypeptide
QSVLTQPPSASGTPGQRVTISCSGSSSNIGSNYVYWYQQLPGTAPKLLIYRNNQRPSGVPDRFSGSKSGTSASLAISGLRSEDEADYYCAAWDDSLSGPVFGGGTKVTVLGEGKSSGSGSESKASEVQLVQSGAVVKKPGASVKVSCKASGYTFTKYGISWVRQAPEQGLEWMGWISAYNVDTKYAQKFQGRVTMTTDTSTSTAYMELRSLRSDDTAVYYCARRGLDYWGQGTLVTVSS

SEQ ID NO: 189 - protein, 538 aa, synthetic construct
  REGION 1..538: note = Description of Artificial Sequence: Synthetic polypeptide
GDEMGTGTQSALTQPASVSGSPGQSITISCTGTSSDVGGYKSVSWYQQHPGKAPKLMIYDVSNRPSGVSDRFSGSKSGNTASLTISGLQAEDEADYYCSSYTSSSSLWVFGGGTKLTVLGEGKSSGSGSESKASQVQLVQSGAEVKKPGSSVKVSCKASGGTFSSYAISWVRQAPGQGLEWMGRIIPILGIANYAQKFQGRVTMTEDTSTDTAYMELSSLRSEDTAVYYCATDLWGVGADWGQGTLVTVSSSGGGGSGGGGSSGSGGGGDGGGGSGGTDIQMTQSPSSLSASVGDRVTITCRASQSISSYLNWYQQKPGKAPKLLIYAASSLQSGVPSRFSGSGSGTDFTLTISSLQPEDFATYYCQQSYSTPRTFGQGTKVDIKEGKSSGSGSESKASQVQLQESGPGLVKPSQTLSLTCTVSGGSISSDDYYWSWIRQTPGKGLEWIGYIYYSGITYYNPSLKSRVTISVDTSKNQFSLKLSSVTAADTAVYYCAREGCNDGVCYNGVFDYWGQGTLVTVSSSGGGGSHHHHHHHH

SEQ ID NO: 190 - protein, 546 aa, synthetic construct
  REGION 1..546: note = Description of Artificial Sequence: Synthetic polypeptide
GDEMGTGTDIQMTQSPSSLSASVGDRVTITCRASQSISSYLNWYQQKPGKAPKLLIYAASSLQSGVPSRFSGSGSGTDFTLTISSLQPEDFATYYCQQSYSTPRTFGQGTKVDIKEGKSSGSGSESKASQVQLQESGPGLVKPSQTLSLTCTVSGGSISSDDYYWSWIRQTPGKGLEWIGYIYYSGITYYNPSLKSRVTISVDTSKNQFSLKLSSVTAADTAVYYCAREGCNDGVCYNGVFDYWGQGTLVTVSSSGGSGGGGSSGGGGSGGGGSSGGGGDGGGGSGGTQSALTQPASVSGSPGQSITISCTGTSSDVGGYKSVSWYQQHPGKAPKLMIYDVSNRPSGVSDRFSGSKSGNTASLTISGLQAEDEADYYCSSYTSSSSLWVFGGGTKLTVLGEGKSSGSGSESKASQVQLVQSGAEVKKPGSSVKVSCKASGGTFSSYAISWVRQAPGQGLEWMGRIIPILGIANYAQKFQGRVTMTEDTSTDTAYMELSSLRSEDTAVYYCATDLWGVGADWGQGTLVTVSSSSGGGGSHHHHHHHH

SEQ ID NO: 191 - protein, 547 aa, synthetic construct
  REGION 1..547: note = Description of Artificial Sequence: Synthetic polypeptide
GDEMGTGTQSALTQPASVSGSPGQSITISCTGTSSDVGGYKSVSWYQQHPGKAPKLMIYDVSNRPSGVSDRFSGSKSGNTASLTISGLQAEDEADYYCSSYTSSSSLWVFGGGTKLTVLGEGKSSGSGSESKASQVQLVQSGAEVKKPGSSVKVSCKASGGTFSSYAISWVRQAPGQGLEWMGRIIPILGIANYAQKFQGRVTMTEDTSTDTAYMELSSLRSEDTAVYYCATDLWGVGADWGQGTLVTVSSSGGGGSGGGGSSGGGGSGGGGSSGGGGDGGGGSGGTDIQMTQSPSSLSASVGDRVTITCRASQSISSYLNWYQQKPGKAPKLLIYAASSLQSGVPSRFSGSGSGTDFTLTISSLQPEDFATYYCQQSYSTPRTFGQGTKVDIKEGKSSGSGSESKASQVQLQESGPGLVKPSQTLSLTCTVSGGSISSDDYYWSWIRQTPGKGLEWIGYIYYSGITYYNPSLKSRVTISVDTSKNQFSLKLSSVTAADTAVYYCAREGCNDGVCYNGVFDYWGQGTLVTVSSSGGGGSHHHHHHHH

SEQ ID NO: 192 - protein, 25 aa, synthetic construct
  REGION 1..25: note = Description of Artificial Sequence: Synthetic peptide
SGGGGSGGGGSSGSGGGGDGGGGSG

SEQ ID NO: 193 - protein, 32 aa, synthetic construct
  REGION 1..32: note = Description of Artificial Sequence: Synthetic polypeptide
SGGSGGGGSSGGGGSGGGGSSGGGGDGGGGSG

SEQ ID NO: 194 - protein, 13 aa, synthetic construct
  REGION 1..13: note = Description of Artificial Sequence: Synthetic peptide
GSGGGGDGGGGSG

SEQ ID NO: 195 - protein, 25 aa, synthetic construct
  REGION 1..25: note = Description of Artificial Sequence: Synthetic peptide
GSGGGGDSGGGGSGGGGSSGGGGSG

SEQ ID NO: 196 - protein, 32 aa, synthetic construct
  REGION 1..32: note = Description of Artificial Sequence: Synthetic polypeptide
GSGGGGDSGGGGSGGSGGSGGSGGGSGGGGSG

SEQ ID NO: 197 - protein, 227 aa, synthetic construct
  REGION 1..227: note = Description of Artificial Sequence: Synthetic polypeptide
DKTHTCPPCPAPELLGGPSVFLFPPKPKDTLMISRTPEVTCVVVDVSHEDPEVKFNWYVDGVEVHNAKTKPREEQYNSTYRVVSVLTVLHQDWLNGKEYKCKVSNKALPAPIEKTISKAKGQPREPQVYTLPPSREELTKNQVSLTCLVKGFYPSDIAVEWESNGQPENNYKTTPPVLDSDGSFFLYSKLTVDKSRWQQGNVFSCSVMHEALHNHYTQKSLSLSPGS

SEQ ID NO: 198 - protein, 12 aa, synthetic construct
  REGION 1..12: note = Description of Artificial Sequence: Synthetic peptide
GGHHHHHHHHGG

SEQ ID NO: 199 - protein, 20 aa, synthetic construct
  REGION 1..20: note = Description of Artificial Sequence: Synthetic peptide
SGGGGSHHHHHHHHSGGGGS

SEQ ID NO: 200 - protein, 24 aa, synthetic construct
  REGION 1..24: note = Description of Artificial Sequence: Synthetic peptide
SGGGGSGGHHHHHHHHGGSGGGGS

SEQ ID NO: 201 - protein, 762 aa, synthetic construct
  REGION 1..762: note = Description of Artificial Sequence: Synthetic polypeptide
GDEMGTQSALTQPASVSGSPGQSITISCTGTSSDVGGYKSVSWYQQHPGKAPKLMIYDVSNRPSGVSDRFSGSKSGNTASLTISGLQAEDEADYYCSSYTSSSSLWVFGGGTKLTVLGEGKSSGSGSESKASQVQLVQSGAEVKKPGSSVKVSCKASGGTFSSYAISWVRQAPGQGLEWMGRIIPILGIANYAQKFQGRVTMTEDTSTDTAYMELSSLRSEDTAVYYCATDLWGVGADWGQGTLVTVSSSGGGGSGGGGSSGSGGGGDGGGGSGGTDIQMTQSPSSLSASVGDRVTITCRASQSISSYLNWYQQKPGKAPKLLIYAASSLQSGVPSRFSGSGSGTDFTLTISSLQPEDFATYYCQQSYSTPRTFGQGTKVDIKEGKSSGSGSESKASQVQLQESGPGLVKPSQTLSLTCTVSGGSISSDDYYWSWIRQTPGKGLEWIGYIYYSGITYYNPSLKSRVTISVDTSKNQFSLKLSSVTAADTAVYYCAREGCNDGVCYNGVFDYWGQGTLVTVSSGSGGGGDGGGGSGDKTHTCPPCPAPELLGGPSVFLFPPKPKDTLMISRTPEVTCVVVDVSHEDPEVKFNWYVDGVEVHNAKTKPREEQYNSTYRVVSVLTVLHQDWLNGKEYKCKVSNKALPAPIEKTISKAKGQPREPQVYTLPPSREELTKNQVSLTCLVKGFYPSDIAVEWESNGQPENNYKTTPPVLDSDGSFFLYSKLTVDKSRWQQGNVFSCSVMHEALHNHYTQKSLSLSPGS

SEQ ID NO: 202 - protein, 774 aa, synthetic construct
  REGION 1..774: note = Description of Artificial Sequence: Synthetic polypeptide
GDEMGTQSALTQPASVSGSPGQSITISCTGTSSDVGGYKSVSWYQQHPGKAPKLMIYDVSNRPSGVSDRFSGSKSGNTASLTISGLQAEDEADYYCSSYTSSSSLWVFGGGTKLTVLGEGKSSGSGSESKASQVQLVQSGAEVKKPGSSVKVSCKASGGTFSSYAISWVRQAPGQGLEWMGRIIPILGIANYAQKFQGRVTMTEDTSTDTAYMELSSLRSEDTAVYYCATDLWGVGADWGQGTLVTVSSSGGGGSGGGGSSGSGGGGDGGGGSGGTDIQMTQSPSSLSASVGDRVTITCRASQSISSYLNWYQQKPGKAPKLLIYAASSLQSGVPSRFSGSGSGTDFTLTISSLQPEDFATYYCQQSYSTPRTFGQGTKVDIKEGKSSGSGSESKASQVQLQESGPGLVKPSQTLSLTCTVSGGSISSDDYYWSWIRQTPGKGLEWIGYIYYSGITYYNPSLKSRVTISVDTSKNQFSLKLSSVTAADTAVYYCAREGCNDGVCYNGVFDYWGQGTLVTVSSGSGGGGDSGGGGSGGGGSSGGGGSGDKTHTCPPCPAPELLGGPSVFLFPPKPKDTLMISRTPEVTCVVVDVSHEDPEVKFNWYVDGVEVHNAKTKPREEQYNSTYRVVSVLTVLHQDWLNGKEYKCKVSNKALPAPIEKTISKAKGQPREPQVYTLPPSREELTKNQVSLTCLVKGFYPSDIAVEWESNGQPENNYKTTPPVLDSDGSFFLYSKLTVDKSRWQQGNVFSCSVMHEALHNHYTQKSLSLSPGS

SEQ ID NO: 203 - protein, 781 aa, synthetic construct
  REGION 1..781: note = Description of Artificial Sequence: Synthetic polypeptide
GDEMGTQSALTQPASVSGSPGQSITISCTGTSSDVGGYKSVSWYQQHPGKAPKLMIYDVSNRPSGVSDRFSGSKSGNTASLTISGLQAEDEADYYCSSYTSSSSLWVFGGGTKLTVLGEGKSSGSGSESKASQVQLVQSGAEVKKPGSSVKVSCKASGGTFSSYAISWVRQAPGQGLEWMGRIIPILGIANYAQKFQGRVTMTEDTSTDTAYMELSSLRSEDTAVYYCATDLWGVGADWGQGTLVTVSSSGGGGSGGGGSSGSGGGGDGGGGSGGTDIQMTQSPSSLSASVGDRVTITCRASQSISSYLNWYQQKPGKAPKLLIYAASSLQSGVPSRFSGSGSGTDFTLTISSLQPEDFATYYCQQSYSTPRTFGQGTKVDIKEGKSSGSGSESKASQVQLQESGPGLVKPSQTLSLTCTVSGGSISSDDYYWSWIRQTPGKGLEWIGYIYYSGITYYNPSLKSRVTISVDTSKNQFSLKLSSVTAADTAVYYCAREGCNDGVCYNGVFDYWGQGTLVTVSSGSGGGGDSGGGGSGGSGGSGGSGGGSGGGGSGDKTHTCPPCPAPELLGGPSVFLFPPKPKDTLMISRTPEVTCVVVDVSHEDPEVKFNWYVDGVEVHNAKTKPREEQYNSTYRVVSVLTVLHQDWLNGKEYKCKVSNKALPAPIEKTISKAKGQPREPQVYTLPPSREELTKNQVSLTCLVKGFYPSDIAVEWESNGQPENNYKTTPPVLDSDGSFFLYSKLTVDKSRWQQGNVFSCSVMHEALHNHYTQKSLSLSPGS

SEQ ID NO: 204 - protein, 769 aa, synthetic construct
  REGION 1..769: note = Description of Artificial Sequence: Synthetic polypeptide
GDEMGTDIQMTQSPSSLSASVGDRVTITCRASQSISSYLNWYQQKPGKAPKLLIYAASSLQSGVPSRFSGSGSGTDFTLTISSLQPEDFATYYCQQSYSTPRTFGQGTKVDIKEGKSSGSGSESKASQVQLQESGPGLVKPSQTLSLTCTVSGGSISSDDYYWSWIRQTPGKGLEWIGYIYYSGITYYNPSLKSRVTISVDTSKNQFSLKLSSVTAADTAVYYCAREGCNDGVCYNGVFDYWGQGTLVTVSSSGGSGGGGSSGGGGSGGGGSSGGGGDGGGGSGGTQSALTQPASVSGSPGQSITISCTGTSSDVGGYKSVSWYQQHPGKAPKLMIYDVSNRPSGVSDRFSGSKSGNTASLTISGLQAEDEADYYCSSYTSSSSLWVFGGGTKLTVLGEGKSSGSGSESKASQVQLVQSGAEVKKPGSSVKVSCKASGGTFSSYAISWVRQAPGQGLEWMGRIIPILGIANYAQKFQGRVTMTEDTSTDTAYMELSSLRSEDTAVYYCATDLWGVGADWGQGTLVTVSSGSGGGGDGGGGSGDKTHTCPPCPAPELLGGPSVFLFPPKPKDTLMISRTPEVTCVVVDVSHEDPEVKFNWYVDGVEVHNAKTKPREEQYNSTYRVVSVLTVLHQDWLNGKEYKCKVSNKALPAPIEKTISKAKGQPREPQVYTLPPSREELTKNQVSLTCLVKGFYPSDIAVEWESNGQPENNYKTTPPVLDSDGSFFLYSKLTVDKSRWQQGNVFSCSVMHEALHNHYTQKSLSLSPGS

SEQ ID NO: 205 - protein, 781 aa, synthetic construct
  REGION 1..781: note = Description of Artificial Sequence: Synthetic polypeptide
GDEMGTDIQMTQSPSSLSASVGDRVTITCRASQSISSYLNWYQQKPGKAPKLLIYAASSLQSGVPSRFSGSGSGTDFTLTISSLQPEDFATYYCQQSYSTPRTFGQGTKVDIKEGKSSGSGSESKASQVQLQESGPGLVKPSQTLSLTCTVSGGSISSDDYYWSWIRQTPGKGLEWIGYIYYSGITYYNPSLKSRVTISVDTSKNQFSLKLSSVTAADTAVYYCAREGCNDGVCYNGVFDYWGQGTLVTVSSSGGSGGGGSSGGGGSGGGGSSGGGGDGGGGSGGTQSALTQPASVSGSPGQSITISCTGTSSDVGGYKSVSWYQQHPGKAPKLMIYDVSNRPSGVSDRFSGSKSGNTASLTISGLQAEDEADYYCSSYTSSSSLWVFGGGTKLTVLGEGKSSGSGSESKASQVQLVQSGAEVKKPGSSVKVSCKASGGTFSSYAISWVRQAPGQGLEWMGRIIPILGIANYAQKFQGRVTMTEDTSTDTAYMELSSLRSEDTAVYYCATDLWGVGADWGQGTLVTVSSGSGGGGDSGGGGSGGGGSSGGGGSGDKTHTCPPCPAPELLGGPSVFLFPPKPKDTLMISRTPEVTCVVVDVSHEDPEVKFNWYVDGVEVHNAKTKPREEQYNSTYRVVSVLTVLHQDWLNGKEYKCKVSNKALPAPIEKTISKAKGQPREPQVYTLPPSREELTKNQVSLTCLVKGFYPSDIAVEWESNGQPENNYKTTPPVLDSDGSFFLYSKLTVDKSRWQQGNVFSCSVMHEALHNHYTQKSLSLSPGS

SEQ ID NO: 206 - protein, 788 aa, synthetic construct
  REGION 1..788: note = Description of Artificial Sequence: Synthetic polypeptide
GDEMGTDIQMTQSPSSLSASVGDRVTITCRASQSISSYLNWYQQKPGKAPKLLIYAASSLQSGVPSRFSGSGSGTDFTLTISSLQPEDFATYYCQQSYSTPRTFGQGTKVDIKEGKSSGSGSESKASQVQLQESGPGLVKPSQTLSLTCTVSGGSISSDDYYWSWIRQTPGKGLEWIGYIYYSGITYYNPSLKSRVTISVDTSKNQFSLKLSSVTAADTAVYYCAREGCNDGVCYNGVFDYWGQGTLVTVSSSGGSGGGGSSGGGGSGGGGSSGGGGDGGGGSGGTQSALTQPASVSGSPGQSITISCTGTSSDVGGYKSVSWYQQHPGKAPKLMIYDVSNRPSGVSDRFSGSKSGNTASLTISGLQAEDEADYYCSSYTSSSSLWVFGGGTKLTVLGEGKSSGSGSESKASQVQLVQSGAEVKKPGSSVKVSCKASGGTFSSYAISWVRQAPGQGLEWMGRIIPILGIANYAQKFQGRVTMTEDTSTDTAYMELSSLRSEDTAVYYCATDLWGVGADWGQGTLVTVSSGSGGGGDSGGGGSGGSGGSGGSGGGSGGGGSGDKTHTCPPCPAPELLGGPSVFLFPPKPKDTLMISRTPEVTCVVVDVSHEDPEVKFNWYVDGVEVHNAKTKPREEQYNSTYRVVSVLTVLHQDWLNGKEYKCKVSNKALPAPIEKTISKAKGQPREPQVYTLPPSREELTKNQVSLTCLVKGFYPSDIAVEWESNGQPENNYKTTPPVLDSDGSFFLYSKLTVDKSRWQQGNVFSCSVMHEALHNHYTQKSLSLSPGS

SEQ ID NO: 207 - protein, 1059 aa, synthetic construct
  REGION 1..1059: note = Description of Artificial Sequence: Synthetic polypeptide
GDEMGTQSALTQPASVSGSPGQSITISCTGTSSDVGGYKSVSWYQQHPGKAPKLMIYDVSNRPSGVSDRFSGSKSGNTASLTISGLQAEDEADYYCSSYTSSSSLWVFGGGTKLTVLGEGKSSGSGSESKASQVQLVQSGAEVKKPGSSVKVSCKASGGTFSSYAISWVRQAPGQGLEWMGRIIPILGIANYAQKFQGRVTMTEDTSTDTAYMELSSLRSEDTAVYYCATDLWGVGADWGQGTLVTVSSSGGGGSGGGGSSGSGGGGDGGGGSGGTDIQMTQSPSSLSASVGDRVTITCRASQSISSYLNWYQQKPGKAPKLLIYAASSLQSGVPSRFSGSGSGTDFTLTISSLQPEDFATYYCQQSYSTPRTFGQGTKVDIKEGKSSGSGSESKASQVQLQESGPGLVKPSQTLSLTCTVSGGSISSDDYYWSWIRQTPGKGLEWIGYIYYSGITYYNPSLKSRVTISVDTSKNQFSLKLSSVTAADTAVYYCAREGCNDGVCYNGVFDYWGQGTLVTVSSGGHHHHHHHHGGGTDIQMTQSPSSLSASVGDRVTITCRASQSISSYLNWYQQKPGKAPKLLIYAASSLQSGVPSRFSGSGSGTDFTLTISSLQPEDFATYYCQQSYSTPRTFGQGTKVDIKEGKSSGSGSESKASQVQLQESGPGLVKPSQTLSLTCTVSGGSISSDDYYWSWIRQTPGKGLEWIGYIYYSGITYYNPSLKSRVTISVDTSKNQFSLKLSSVTAADTAVYYCAREGCNDGVCYNGVFDYWGQGTLVTVSSSGGSGGGGSSGGGGSGGGGSSGGGGDGGGGSGGTQSALTQPASVSGSPGQSITISCTGTSSDVGGYKSVSWYQQHPGKAPKLMIYDVSNRPSGVSDRFSGSKSGNTASLTISGLQAEDEADYYCSSYTSSSSLWVFGGGTKLTVLGEGKSSGSGSESKASQVQLVQSGAEVKKPGSSVKVSCKASGGTFSSYAISWVRQAPGQGLEWMGRIIPILGIANYAQKFQGRVTMTEDTSTDTAYMELSSLRSEDTAVYYCATDLWGVGADWGQGTLVTVSS

SEQ ID NO: 208 - protein, 1067 aa, synthetic construct
  REGION 1..1067: note = Description of Artificial Sequence: Synthetic polypeptide
GDEMGTQSALTQPASVSGSPGQSITISCTGTSSDVGGYKSVSWYQQHPGKAPKLMIYDVSNRPSGVSDRFSGSKSGNTASLTISGLQAEDEADYYCSSYTSSSSLWVFGGGTKLTVLGEGKSSGSGSESKASQVQLVQSGAEVKKPGSSVKVSCKASGGTFSSYAISWVRQAPGQGLEWMGRIIPILGIANYAQKFQGRVTMTEDTSTDTAYMELSSLRSEDTAVYYCATDLWGVGADWGQGTLVTVSSSGGGGSGGGGSSGSGGGGDGGGGSGGTDIQMTQSPSSLSASVGDRVTITCRASQSISSYLNWYQQKPGKAPKLLIYAASSLQSGVPSRFSGSGSGTDFTLTISSLQPEDFATYYCQQSYSTPRTFGQGTKVDIKEGKSSGSGSESKASQVQLQESGPGLVKPSQTLSLTCTVSGGSISSDDYYWSWIRQTPGKGLEWIGYIYYSGITYYNPSLKSRVTISVDTSKNQFSLKLSSVTAADTAVYYCAREGCNDGVCYNGVFDYWGQGTLVTVSSSGGGGSHHHHHHHHSGGGGSGTDIQMTQSPSSLSASVGDRVTITCRASQSISSYLNWYQQKPGKAPKLLIYAASSLQSGVPSRFSGSGSGTDFTLTISSLQPEDFATYYCQQSYSTPRTFGQGTKVDIKEGKSSGSGSESKASQVQLQESGPGLVKPSQTLSLTCTVSGGSISSDDYYWSWIRQTPGKGLEWIGYIYYSGITYYNPSLKSRVTISVDTSKNQFSLKLSSVTAADTAVYYCAREGCNDGVCYNGVFDYWGQGTLVTVSSSGGSGGGGSSGGGGSGGGGSSGGGGDGGGGSGGTQSALTQPASVSGSPGQSITISCTGTSSDVGGYKSVSWYQQHPGKAPKLMIYDVSNRPSGVSDRFSGSKSGNTASLTISGLQAEDEADYYCSSYTSSSSLWVFGGGTKLTVLGEGKSSGSGSESKASQVQLVQSGAEVKKPGSSVKVSCKASGGTFSSYAISWVRQAPGQGLEWMGRIIPILGIANYAQKFQGRVTMTEDTSTDTAYMELSSLRSEDTAVYYCATDLWGVGADWGQGTLVTVSS

SEQ ID NO: 209 - protein, 1071 aa, synthetic construct
  REGION 1..1071: note = Description of Artificial Sequence: Synthetic polypeptide
GDEMGTQSALTQPASVSGSPGQSITISCTGTSSDVGGYKSVSWYQQHPGKAPKLMIYDVSNRPSGVSDRFSGSKSGNTASLTISGLQAEDEADYYCSSYTSSSSLWVFGGGTKLTVLGEGKSSGSGSESKASQVQLVQSGAEVKKPGSSVKVSCKASGGTFSSYAISWVRQAPGQGLEWMGRIIPILGIANYAQKFQGRVTMTEDTSTDTAYMELSSLRSEDTAVYYCATDLWGVGADWGQGTLVTVSSSGGGGSGGGGSSGSGGGGDGGGGSGGTDIQMTQSPSSLSASVGDRVTITCRASQSISSYLNWYQQKPGKAPKLLIYAASSLQSGVPSRFSGSGSGTDFTLTISSLQPEDFATYYCQQSYSTPRTFGQGTKVDIKEGKSSGSGSESKASQVQLQESGPGLVKPSQTLSLTCTVSGGSISSDDYYWSWIRQTPGKGLEWIGYIYYSGITYYNPSLKSRVTISVDTSKNQFSLKLSSVTAADTAVYYCAREGCNDGVCYNGVFDYWGQGTLVTVSSSGGGGSGGHHHHHHHHGGSGGGGSGTDIQMTQSPSSLSASVGDRVTITCRASQSISSYLNWYQQKPGKAPKLLIYAASSLQSGVPSRFSGSGSGTDFTLTISSLQPEDFATYYCQQSYSTPRTFGQGTKVDIKEGKSSGSGSESKASQVQLQESGPGLVKPSQTLSLTCTVSGGSISSDDYYWSWIRQTPGKGLEWIGYIYYSGITYYNPSLKSRVTISVDTSKNQFSLKLSSVTAADTAVYYCAREGCNDGVCYNGVFDYWGQGTLVTVSSSGGSGGGGSSGGGGSGGGGSSGGGGDGGGGSGGTQSALTQPASVSGSPGQSITISCTGTSSDVGGYKSVSWYQQHPGKAPKLMIYDVSNRPSGVSDRFSGSKSGNTASLTISGLQAEDEADYYCSSYTSSSSLWVFGGGTKLTVLGEGKSSGSGSESKASQVQLVQSGAEVKKPGSSVKVSCKASGGTFSSYAISWVRQAPGQGLEWMGRIIPILGIANYAQKFQGRVTMTEDTSTDTAYMELSSLRSEDTAVYYCATDLWGVGADWGQGTLVTVSS

SEQ ID NO: 210 - protein, 1050 aa, synthetic construct
  REGION 1..1050: note = Description of Artificial Sequence: Synthetic polypeptide
GDEMGTQSALTQPASVSGSPGQSITISCTGTSSDVGGYKSVSWYQQHPGKAPKLMIYDVSNRPSGVSDRFSGSKSGNTASLTISGLQAEDEADYYCSSYTSSSSLWVFGGGTKLTVLGEGKSSGSGSESKASQVQLVQSGAEVKKPGSSVKVSCKASGGTFSSYAISWVRQAPGQGLEWMGRIIPILGIANYAQKFQGRVTMTEDTSTDTAYMELSSLRSEDTAVYYCATDLWGVGADWGQGTLVTVSSSGGGGSGGGGSSGSGGGGDGGGGSGGTDIQMTQSPSSLSASVGDRVTITCRASQSISSYLNWYQQKPGKAPKLLIYAASSLQSGVPSRFSGSGSGTDFTLTISSLQPEDFATYYCQQSYSTPRTFGQGTKVDIKEGKSSGSGSESKASQVQLQESGPGLVKPSQTLSLTCTVSGGSISSDDYYWSWIRQTPGKGLEWIGYIYYSGITYYNPSLKSRVTISVDTSKNQFSLKLSSVTAADTAVYYCAREGCNDGVCYNGVFDYWGQGTLVTVSSGGHHHHHHHHGGGTDIQMTQSPSSLSASVGDRVTITCRASQSISSYLNWYQQKPGKAPKLLIYAASSLQSGVPSRFSGSGSGTDFTLTISSLQPEDFATYYCQQSYSTPRTFGQGTKVDIKEGKSSGSGSESKASQVQLQESGPGLVKPSQTLSLTCTVSGGSISSDDYYWSWIRQTPGKGLEWIGYIYYSGITYYNPSLKSRVTISVDTSKNQFSLKLSSVTAADTAVYYCAREGCNDGVCYNGVFDYWGQGTLVTVSSSGGSGGGGSSGSGGGGDGGGGSGGTQSALTQPASVSGSPGQSITISCTGTSSDVGGYKSVSWYQQHPGKAPKLMIYDVSNRPSGVSDRFSGSKSGNTASLTISGLQAEDEADYYCSSYTSSSSLWVFGGGTKLTVLGEGKSSGSGSESKASQVQLVQSGAEVKKPGSSVKVSCKASGGTFSSYAISWVRQAPGQGLEWMGRIIPILGIANYAQKFQGRVTMTEDTSTDTAYMELSSLRSEDTAVYYCATDLWGVGADWGQGTLVTVSS

SEQ ID NO: 211 - DNA, 894 bp, synthetic construct
  misc_feature 1..894: note = Description of Artificial Sequence: Synthetic polynucleotide
  modified_base 861: mod_base = OTHER; note = a, c, t, g, unknown or other
  modified_base 872: mod_base = OTHER; note = a, c, t, g, unknown or other
  source 1..894: mol_type = other DNA
gacgacgatgacaagcttcaggctgtgctcactcagccgtcttccctctctgcatctcctggagcttcagccagtctcacctgcaccttacacagtggcatcaatgttgctacctacaggatatactggtaccagcagaagccagggagtcctccccagtatctgctgacttataagtcagacttagataaacatcaggggtctggagtccccagtcgcttctctggatccaaagatgcgtcggccaatgcaggcatattgctcatttctggactccagtctgacgacgagggtgactattattgtttaatctggcacgactacgtctggtacttcggcggtgggaccaaggtcaccgtcctaggtgagggtaaatcgtccggatctggttccgaatccaaagctagcgaggtgcagctgttggagtctgggggaggcttggtacagcctggcaggtccctgagactctcctgtgcagcctctggattcacctttgatgattatgccatgcactgggtccggcaagctccagggaagggcctggagtgggtctcaggtattagttggaatagtggtagcataggctatgcggactctgtgaagggccgattcaccatctccagagacaacgccaagaactccctgtatctgcaaatgaacagtctgagagctgaggacacggctctgtattattgtgcaaaaggcgggtggggcagctcgacccactactactacggtatggacgtctggggccaagggaccacggtcaccgtctcctcagtcgacccattcgtttctgaatatcaaggccaatcgtctgacctgcctcaacctcctgtcaatgctggcggcggctctganggaggcgggtnccggtggtggctctggttccgg

SEQ ID NO: 212 - protein, 298 aa, synthetic construct
  REGION 1..298: note = Description of Artificial Sequence: Synthetic polypeptide
  MOD_RES 287: note = Any amino acid
  MOD_RES 291: note = Any amino acid
DDDDKLQAVLTQPSSLSASPGASASLTCTLHSGINVATYRIYWYQQKPGSPPQYLLTYKSDLDKHQGSGVPSRFSGSKDASANAGILLISGLQSDDEGDYYCLIWHDYVWYFGGGTKVTVLGEGKSSGSGSESKASEVQLLESGGGLVQPGRSLRLSCAASGFTFDDYAMHWVRQAPGKGLEWVSGISWNSGSIGYADSVKGRFTISRDNAKNSLYLQMNSLRAEDTALYYCAKGGWGSSTHYYYGMDVWGQGTTVTVSSVDPFVSEYQGQSSDLPQPPVNAGGGSXGGGXRWWLWFR

SEQ ID NO: 213 - protein, 11 aa, synthetic construct
  REGION 1..11: note = Description of Artificial Sequence: Synthetic peptide
AAWDDSLNGRV

SEQ ID NO: 214 - protein, 5 aa, synthetic construct
  REGION 1..5: note = Description of Artificial Sequence: Synthetic peptide
IYAMS

SEQ ID NO: 215 - protein, 17 aa, synthetic construct
  REGION 1..17: note = Description of Artificial Sequence: Synthetic peptide
AISGSGGSTYYADSVKG

SEQ ID NO: 216 - protein, 4 aa, synthetic construct
  REGION 1..4: note = Description of Artificial Sequence: Synthetic peptide
DFDY

SEQ ID NO: 217 - protein, 13 aa, synthetic construct
  REGION 1..13: note = Description of Artificial Sequence: Synthetic peptide
SGSSSNIGSNYVY

SEQ ID NO: 218 - protein, 7 aa, synthetic construct
  REGION 1..7: note = Description of Artificial Sequence: Synthetic peptide
GNINRPS

SEQ ID NO: 219 - protein, 11 aa, synthetic construct
  REGION 1..11: note = Description of Artificial Sequence: Synthetic peptide
AAWDDSLNGRV

SEQ ID NO: 220 - protein, 5 aa, synthetic construct
  REGION 1..5: note = Description of Artificial Sequence: Synthetic peptide
NAWMN

SEQ ID NO: 221 - protein, 17 aa, synthetic construct
  REGION 1..17: note = Description of Artificial Sequence: Synthetic peptide
SISSSSSYIYYADSVKG

SEQ ID NO: 222 - protein, 13 aa, synthetic construct
  REGION 1..13: note = Description of Artificial Sequence: Synthetic peptide
AVAAGGMFWGLDQ

SEQ ID NO: 223 - protein, 13 aa, synthetic construct
  REGION 1..13: note = Description of Artificial Sequence: Synthetic peptide
SGSRSNIGSNSVH

SEQ ID NO: 224 - protein, 7 aa, synthetic construct
  REGION 1..7: note = Description of Artificial Sequence: Synthetic peptide
GNSNRPS

SEQ ID NO: 225 - protein, 12 aa, synthetic construct
  REGION 1..12: note = Description of Artificial Sequence: Synthetic peptide
QSYDSSLNDHVV

SEQ ID NO: 226 - protein, 5 aa, synthetic construct
  REGION 1..5: note = Description of Artificial Sequence: Synthetic peptide
DYYMT

SEQ ID NO: 227 - protein, 15 aa, synthetic construct
  REGION 1..15: note = Description of Artificial Sequence: Synthetic peptide
SISGGSTYYADSRKG

SEQ ID NO: 228 - protein, 15 aa, synthetic construct
  REGION 1..15: note = Description of Artificial Sequence: Synthetic peptide
DFGVAGWFGQYGMDV

SEQ ID NO: 229 - protein, 14 aa, synthetic construct
  REGION 1..14: note = Description of Artificial Sequence: Synthetic peptide
TGSSSNIGAGYDVH

SEQ ID NO: 230 - protein, 7 aa, synthetic construct
  REGION 1..7: note = Description of Artificial Sequence: Synthetic peptide
RSNQRPS

SEQ ID NO: 231 - protein, 10 aa, synthetic construct
  REGION 1..10: note = Description of Artificial Sequence: Synthetic peptide
SSYAGNYNLV

SEQ ID NO: 232 - protein, 5 aa, synthetic construct
  REGION 1..5: note = Description of Artificial Sequence: Synthetic peptide
SYAMS

SEQ ID NO: 233 - protein, 17 aa, synthetic construct
  REGION 1..17: note = Description of Artificial Sequence: Synthetic peptide
NINQDGSEKNYVDSMRG

SEQ ID NO: 234 - protein, 4 aa, synthetic construct
  REGION 1..4: note = Description of Artificial Sequence: Synthetic peptide
EFDY

SEQ ID NO: 235 - protein, 7 aa, synthetic construct
  REGION 1..7: note = Description of Artificial Sequence: Synthetic peptide
GNNKRPS

SEQ ID NO: 236 - protein, 16 aa, synthetic construct
  REGION 1..16: note = Description of Artificial Sequence: Synthetic peptide
NINQDGSEKNYVDSMR

SEQ ID NO: 237 - protein, 7 aa, synthetic construct
  REGION 1..7: note = Description of Artificial Sequence: Synthetic peptide
GYTFTGY

SEQ ID NO: 238 - protein, 10 aa, synthetic construct
  REGION 1..10: note = Description of Artificial Sequence: Synthetic peptide
GYTFTGYYMH

SEQ ID NO: 239 - protein, 5 aa, synthetic construct
  REGION 1..5: note = Description of Artificial Sequence: Synthetic peptide
GYYMH

SEQ ID NO: 240 - protein, 6 aa, synthetic construct
  REGION 1..6: note = Description of Artificial Sequence: Synthetic peptide
TGYYMH

SEQ ID NO: 241 - protein, 8 aa, synthetic construct
  REGION 1..8: note = Description of Artificial Sequence: Synthetic peptide
GYTFTGYY

SEQ ID NO: 242 - protein, 6 aa, synthetic construct
  REGION 1..6: note = Description of Artificial Sequence: Synthetic peptide
NPNSGG

SEQ ID NO: 243 - protein, 10 aa, synthetic construct
  REGION 1..10: note = Description of Artificial Sequence: Synthetic peptide
RINPNSGGTN

SEQ ID NO: 244 - protein, 17 aa, synthetic construct
  REGION 1..17: note = Description of Artificial Sequence: Synthetic peptide
RINPNSGGTNYAQKFQG

SEQ ID NO: 245 - protein, 13 aa, synthetic construct
  REGION 1..13: note = Description of Artificial Sequence: Synthetic peptide
WMGRINPNSGGTN

SEQ ID NO: 246 - protein, 8 aa, synthetic construct
  REGION 1..8: note = Description of Artificial Sequence: Synthetic peptide
INPNSGGT

SEQ ID NO: 247 - protein, 13 aa, synthetic construct
  REGION 1..13: note = Description of Artificial Sequence: Synthetic peptide
DPTYYDILTGPEY

SEQ ID NO: 248 - protein, 14 aa, synthetic construct
  REGION 1..14: note = Description of Artificial Sequence: Synthetic peptide
ARDPTYYDILTGPE

SEQ ID NO: 249 - protein, 15 aa, synthetic construct
  REGION 1..15: note = Description of Artificial Sequence: Synthetic peptide
ARDPTYYDILTGPEY

SEQ ID NO: 250 - protein, 14 aa, synthetic construct
  REGION 1..14: note = Description of Artificial Sequence: Synthetic peptide
TGTNTDIGYYNYVS

SEQ ID NO: 251 - protein, 10 aa, synthetic construct
  REGION 1..10: note = Description of Artificial Sequence: Synthetic peptide
IGYYNYVSWY

SEQ ID NO: 252 - protein, 9 aa, synthetic construct
  REGION 1..9: note = Description of Artificial Sequence: Synthetic peptide
NTDIGYYNY

SEQ ID NO: 253 - protein, 7 aa, synthetic construct
  REGION 1..7: note = Description of Artificial Sequence: Synthetic peptide
EVDNRPS

SEQ ID NO: 254 - protein, 10 aa, synthetic construct
  REGION 1..10: note = Description of Artificial Sequence: Synthetic peptide
LLIFEVDNRP

SEQ ID NO: 255 - protein, 10 aa, synthetic construct
  REGION 1..10: note = Description of Artificial Sequence: Synthetic peptide
SSYSTYNILL

SEQ ID NO: 256 - protein, 121 aa, synthetic construct
  REGION 1..121: note = Description of Artificial Sequence: Synthetic polypeptide
EVQLLESEAEVKKPGASVKVSCKASGYTFTGYYMHWVRQAPGQGLEWMGRINPNSGGTNYAQKFQGRVTMTRDTSISTAYMELSRLRSDDTAVYYCARDPTYYDILTGPEYWGQGTVTVSS

SEQ ID NO: 257 - protein, 111 aa, synthetic construct
  REGION 1..111: note = Description of Artificial Sequence: Synthetic polypeptide
LPVLTQPASVSGSPGQSITFSCTGTNTDIGYYNYVSWYQQLPGKAPKLLIFEVDNRPSGVPSRFSGSKSGNTASLTISGLQAEDEADYYCSSYSTYNILLFGGGTKLTVLG

SEQ ID NO: 258 - protein, 7 aa, synthetic construct
  REGION 1..7: note = Description of Artificial Sequence: Synthetic peptide
GYNFAGY

SEQ ID NO: 259 - protein, 10 aa, synthetic construct
  REGION 1..10: note = Description of Artificial Sequence: Synthetic peptide
GYNFAGYYVH

SEQ ID NO: 260 - protein, 5 aa, synthetic construct
  REGION 1..5: note = Description of Artificial Sequence: Synthetic peptide
GYYVH

SEQ ID NO: 261 - protein, 6 aa, synthetic construct
  REGION 1..6: note = Description of Artificial Sequence: Synthetic peptide
AGYYVH

SEQ ID NO: 262 - protein, 8 aa, synthetic construct
  REGION 1..8: note = Description of Artificial Sequence: Synthetic peptide
GYNFAGYY

SEQ ID NO: 263 - protein, 10 aa, synthetic construct
  REGION 1..10: note = Description of Artificial Sequence: Synthetic peptide
WINPNSGGTD

SEQ ID NO: 264 - protein, 17 aa, synthetic construct
  REGION 1..17: note = Description of Artificial Sequence: Synthetic peptide
WINPNSGGTDYAQKFQG

SEQ ID NO: 265 - protein, 13 aa, synthetic construct
  REGION 1..13: note = Description of Artificial Sequence: Synthetic peptide
WMGWINPNSGGTD

SEQ ID NO: 266 - protein, 4 aa, synthetic construct
  REGION 1..4: note = Description of Artificial Sequence: Synthetic peptide
NLQF

SEQ ID NO: 267 - protein, 5 aa, synthetic construct
  REGION 1..5: note = Description of Artificial Sequence: Synthetic peptide
ARNLQ

SEQ ID NO: 268 - protein, 6 aa, synthetic construct
  REGION 1..6: note = Description of Artificial Sequence: Synthetic peptide
ARNLQF

SEQ ID NO: 269 - protein, 11 aa, synthetic construct
  REGION 1..11: note = Description of Artificial Sequence: Synthetic peptide
RASQSVSSNLA

SEQ ID NO: 270 - protein, 7 aa, synthetic construct
  REGION 1..7: note = Description of Artificial Sequence: Synthetic peptide
SSNLAWY

SEQ ID NO: 271 - protein, 6 aa, synthetic construct
  REGION 1..6: note = Description of Artificial Sequence: Synthetic peptide
QSVSSN

SEQ ID NO: 272 - protein, 7 aa, synthetic construct
  REGION 1..7: note = Description of Artificial Sequence: Synthetic peptide
GASSRAT

SEQ ID NO: 273 - protein, 10 aa, synthetic construct
  REGION 1..10: note = Description of Artificial Sequence: Synthetic peptide
LLIYGASSRA

SEQ ID NO: 274 - protein, 9 aa, synthetic construct
  REGION 1..9: note = Description of Artificial Sequence: Synthetic peptide
QQYIYSPYT

SEQ ID NO: 275 - protein, 113 aa, synthetic construct
  REGION 1..113: note = Description of Artificial Sequence: Synthetic polypeptide
EVQLVQSGAEVKKPGASVKVSCKASGYNFAGYYVHWVRQAPGQGLEWMGWINPNSGGTDYAQKFQGRVTMTRDTSISTAYMDLSRLRSDDTAVYYCARNLQFFRPGTLVTVSS

SEQ ID NO: 276 - protein, 107 aa, synthetic construct
  REGION 1..107: note = Description of Artificial Sequence: Synthetic polypeptide
EIVMTQSPATLSVSPGERATLSCRASQSVSSNLAWYQQKPGQAPRLLIYGASSRATGIPDRFSGSGSGTDFTLTISRLEPEDFAVYYCQQYIYSPYTFGQGTKVDIK

SEQ ID NO: 277 - protein, 9 aa, synthetic construct
  REGION 1..9: note = Description of Artificial Sequence: Synthetic peptide
GGSISSSSY

SEQ ID NO: 278 - protein, 12 aa, synthetic construct
  REGION 1..12: note = Description of Artificial Sequence: Synthetic peptide
GGSISSSSYYWG

SEQ ID NO: 279 - protein, 7 aa, synthetic construct
  REGION 1..7: note = Description of Artificial Sequence: Synthetic peptide
SSSYYWG

SEQ ID NO: 280 - protein, 8 aa, synthetic construct
  REGION 1..8: note = Description of Artificial Sequence: Synthetic peptide
SSSSYYWG

SEQ ID NO: 281 - protein, 10 aa, synthetic construct
  REGION 1..10: note = Description of Artificial Sequence: Synthetic peptide
GGSISSSSYY

SEQ ID NO: 282 - protein, 5 aa, synthetic construct
  REGION 1..5: note = Description of Artificial Sequence: Synthetic peptide
YYSGS

SEQ ID NO: 283 - protein, 9 aa, synthetic construct
  REGION 1..9: note = Description of Artificial Sequence: Synthetic peptide
SIYYSGSTY

SEQ ID NO: 284 - protein, 16 aa, synthetic construct
  REGION 1..16: note = Description of Artificial Sequence: Synthetic peptide
SIYYSGSTYYNPSLKS

SEQ ID NO: 285 - protein, 12 aa, synthetic construct
  REGION 1..12: note = Description of Artificial Sequence: Synthetic peptide
WIGSIYYSGSTY

SEQ ID NO: 286 - protein, 7 aa, synthetic construct
  REGION 1..7: note = Description of Artificial Sequence: Synthetic peptide
IYYSGST

SEQ ID NO: 287 - protein, 8 aa, synthetic construct
  REGION 1..8: note = Description of Artificial Sequence: Synthetic peptide
QVGPVLKS

SEQ ID NO: 288 - protein, 9 aa, synthetic construct
  REGION 1..9: note = Description of Artificial Sequence: Synthetic peptide
ARQVGPVLK

SEQ ID NO: 289 - protein, 10 aa, synthetic construct
  REGION 1..10: note = Description of Artificial Sequence: Synthetic peptide
ARQVGPVLKS

SEQ ID NO: 290 - protein, 11 aa, synthetic construct
  REGION 1..11: note = Description of Artificial Sequence: Synthetic peptide
GGNNIGSKNVH

SEQ ID NO: 291 - protein, 7 aa, synthetic construct
  REGION 1..7: note = Description of Artificial Sequence: Synthetic peptide
SKNVHWY

SEQ ID NO: 292 - protein, 6 aa, synthetic construct
  REGION 1..6: note = Description of Artificial Sequence: Synthetic peptide
NIGSKN

SEQ ID NO: 293 - protein, 7 aa, synthetic construct
  REGION 1..7: note = Description of Artificial Sequence: Synthetic peptide
DDSDRPS

SEQ ID NO: 294 - protein, 10 aa, synthetic construct
  REGION 1..10: note = Description of Artificial Sequence: Synthetic peptide
LVIYDDSDRP

SEQ ID NO: 295 - protein, 10 aa, synthetic construct
  REGION 1..10: note = Description of Artificial Sequence: Synthetic peptide
QAWDSSTAVV

SEQ ID NO: 296 - protein, 118 aa, synthetic construct
  REGION 1..118: note = Description of Artificial Sequence: Synthetic polypeptide
QVQLQESGPGLVKPSETLSLTCTVSGGSISSSSYYWGWIRQPPGKGLEWIGSIYYSGSTYYNPSLKSRATISVDTSKNQFSLKMTSVTAADTAIYYCARQVGPVLKSVSQGTLVTVTS

SEQ ID NO: 297 - protein, 108 aa, synthetic construct
  REGION 1..108: note = Description of Artificial Sequence: Synthetic polypeptide
SYELTQPLSVSVALGQTARITCGGNNIGSKNVHWYQQKPGQAPVLVIYDDSDRPSGTSERFSGSNSGNTATLTISGTQAMDEADYYCQAWDSSTAVVFGGGTKLTVLG

SEQ ID NO: 298 - protein, 7 aa, synthetic construct
  REGION 1..7: note = Description of Artificial Sequence: Synthetic peptide
GFTFSSY

SEQ ID NO: 299 - protein, 10 aa, synthetic construct
  REGION 1..10: note = Description of Artificial Sequence: Synthetic peptide
GFTFSSYAMS

SEQ ID NO: 300 - protein, 20 aa, synthetic construct
  REGION 1..20: note = Description of Artificial Sequence: Synthetic peptide
GGGGSGGGGSGGGGSGGGGS

SEQ ID NO: 301 - protein, 6 aa, synthetic construct
  REGION 1..6: note = Description of Artificial Sequence: Synthetic peptide
SSYAMS

SEQ ID NO: 302 - protein, 8 aa, synthetic construct
  REGION 1..8: note = Description of Artificial Sequence: Synthetic peptide
GFTFSSYA

SEQ ID NO: 303 - protein, 6 aa, synthetic construct
  REGION 1..6: note = Description of Artificial Sequence: Synthetic peptide
SGSGGS

SEQ ID NO: 304 - protein, 10 aa, synthetic construct
  REGION 1..10: note = Description of Artificial Sequence: Synthetic peptide
AISGSGGSTY

SEQ ID NO: 305 - protein, 13 aa, synthetic construct
  REGION 1..13: note = Description of Artificial Sequence: Synthetic peptide
WVSAISGSGGSTY

SEQ ID NO: 306 - protein, 8 aa, synthetic construct
  REGION 1..8: note = Description of Artificial Sequence: Synthetic peptide
ISGSGGST

SEQ ID NO: 307 - protein, 7 aa, synthetic construct
  REGION 1..7: note = Description of Artificial Sequence: Synthetic peptide
SASFFDY

SEQ ID NO: 308 - protein, 8 aa, synthetic construct
  REGION 1..8: note = Description of Artificial Sequence: Synthetic peptide
AKSASFFD

SEQ ID NO: 309 - protein, 9 aa, synthetic construct
  REGION 1..9: note = Description of Artificial Sequence: Synthetic peptide
AKSASFFDY

SEQ ID NO: 310 - protein, 12 aa, synthetic construct
  REGION 1..12: note = Description of Artificial Sequence: Synthetic peptide
RASQSVSSSYLA

SEQ ID NO: 311 - protein, 8 aa, synthetic construct
  REGION 1..8: note = Description of Artificial Sequence: Synthetic peptide
SSSYLAWY

SEQ ID NO: 312 - protein, 7 aa, synthetic construct
  REGION 1..7: note = Description of Artificial Sequence: Synthetic peptide
QSVSSSY

SEQ ID NO: 313 - protein, 9 aa, synthetic construct
  REGION 1..9: note = Description of Artificial Sequence: Synthetic peptide
QQHFRWPWT

SEQ ID NO: 314 - protein, 116 aa, synthetic construct
  REGION 1..116: note = Description of Artificial Sequence: Synthetic polypeptide
EVQLLESGGGLVQPGGSLRLSCAASGFTFSSYAMSWVRQAPGKGLEWVSAISGSGGSTYYADSVKGRFTISRDNSKNTLYLQMNSLRAEDTAVYYCAKSASFFDYWGQGTLVTVSS

SEQ ID NO: 315 - protein, 108 aa, synthetic construct
  REGION 1..108: note = Description of Artificial Sequence: Synthetic polypeptide
EIVLTQSPGTLSLSPGERATLSCRASQSVSSSYLAWYQQKPGQAPRLLIYGASSRATGIPDRFSGSGSGTDFTLTISRLEPEDFAVYYCQQHFRWPWTFGQGTKVEIK

SEQ ID NO: 316 - protein, 9 aa, synthetic construct
  REGION 1..9: note = Description of Artificial Sequence: Synthetic peptide
GASISSGGY

SEQ ID NO: 317 - protein, 12 aa, synthetic construct
  REGION 1..12: note = Description of Artificial Sequence: Synthetic peptide
GASISSGGYYWS

SEQ ID NO: 318 - protein, 7 aa, synthetic construct
  REGION 1..7: note = Description of Artificial Sequence: Synthetic peptide
SGGYYWS

SEQ ID NO: 319 - protein, 8 aa, synthetic construct
  REGION 1..8: note = Description of Artificial Sequence: Synthetic peptide
SSGGYYWS

SEQ ID NO: 320 - protein, 10 aa, synthetic construct
  REGION 1..10: note = Description of Artificial Sequence: Synthetic peptide
GASISSGGYY

SEQ ID NO: 321 - protein, 9 aa, synthetic construct
  REGION 1..9: note = Description of Artificial Sequence: Synthetic peptide
YSYYSGSTY

SEQ ID NO: 322 - protein, 16 aa, synthetic construct
  REGION 1..16: note = Description of Artificial Sequence: Synthetic peptide
YSYYSGSTYYNPSLKS

SEQ ID NO: 323 - protein, 12 aa, synthetic construct
  REGION 1..12: note = Description of Artificial Sequence: Synthetic peptide
WIGYSYYSGSTY

SEQ ID NO: 324 - protein, 7 aa, synthetic construct
  REGION 1..7: note = Description of Artificial Sequence: Synthetic peptide
SYYSGST

SEQ ID NO: 325 - protein, 7 aa, synthetic construct
  REGION 1..7: note = Description of Artificial Sequence: Synthetic peptide
GGVRFDL

SEQ ID NO: 326 - protein, 8 aa, synthetic construct
  REGION 1..8: note = Description of Artificial Sequence: Synthetic peptide
ARGGVRFD

SEQ ID NO: 327 - protein, 9 aa, synthetic construct
  REGION 1..9: note = Description of Artificial Sequence: Synthetic peptide
ARGGVRFDL

SEQ ID NO: 328 - protein, 13 aa, synthetic construct
  REGION 1..13: note = Description of Artificial Sequence: Synthetic peptide
SGSSSNIGSNTVN

SEQ ID NO: 329 - protein, 9 aa, synthetic construct
  REGION 1..9: note = Description of Artificial Sequence: Synthetic peptide
IGSNTVNWY

SEQ ID NO: 330 - protein, 8 aa, synthetic construct
  REGION 1..8: note = Description of Artificial Sequence: Synthetic peptide
SSNIGSNT

SEQ ID NO: 331 - protein, 7 aa, synthetic construct
  REGION 1..7: note = Description of Artificial Sequence: Synthetic peptide
SNNQRPS

SEQ ID NO: 332 - protein, 10 aa, synthetic construct
  REGION 1..10: note = Description of Artificial Sequence: Synthetic peptide
LLIYSNNQRP

SEQ ID NO: 333 - protein, 11 aa, synthetic construct
  REGION 1..11: note = Description of Artificial Sequence: Synthetic peptide
AAWDDSLNGVV

SEQ ID NO: 334 - protein, 117 aa, synthetic construct
  REGION 1..117: note = Description of Artificial Sequence: Synthetic polypeptide
QVQLQESGPGLVKPSQTLSLTCTVSGASISSGGYYWSWIRQHPGKGLEWIGYSYYSGSTYYNPSLKSRVTISVDTSKNQFSLYLTSVTAADTAVYHCARGGVRFDLWGQGTLVTVSS

SEQ ID NO: 335 - protein, 111 aa, synthetic construct
  REGION 1..111: note = Description of Artificial Sequence: Synthetic polypeptide
SYELTQPPSASGTPGQKVTISCSGSSSNIGSNTVNWYQQLPGTAPKLLIYSNNQRPSGVPDRFSGSKSGTSASLAISGLQSEDEADYYCAAWDDSLNGVVFGGGTKVTVLG

SEQ ID NO: 336 - protein, 23 aa, synthetic construct
  REGION 1..23: note = Description of Artificial Sequence: Synthetic peptide
IPWGDYDFWSGYYTRPGHSGMDV

SEQ ID NO: 337 - protein, 24 aa, synthetic construct
  REGION 1..24: note = Description of Artificial Sequence: Synthetic peptide
AKIPWGDYDFWSGYYTRPGHSGMD

SEQ ID NO: 338 - protein, 25 aa, synthetic construct
  REGION 1..25: note = Description of Artificial Sequence: Synthetic peptide
AKIPWGDYDFWSGYYTRPGHSGMDV

SEQ ID NO: 339 - protein, 11 aa, synthetic construct
  REGION 1..11: note = Description of Artificial Sequence: Synthetic peptide
SGDALPKKYAY

SEQ ID NO: 340 - protein, 7 aa, synthetic construct
  REGION 1..7: note = Description of Artificial Sequence: Synthetic peptide
KKYAYWY

SEQ ID NO: 341 - protein, 6 aa, synthetic construct
  REGION 1..6: note = Description of Artificial Sequence: Synthetic peptide
ALPKKY

SEQ ID NO: 342 - protein, 7 aa, synthetic construct
  REGION 1..7: note = Description of Artificial Sequence: Synthetic peptide
EDSKRPS

SEQ ID NO: 343 - protein, 10 aa, synthetic construct
  REGION 1..10: note = Description of Artificial Sequence: Synthetic peptide
LVIYEDSKRP

SEQ ID NO: 344 - protein, 10 aa, synthetic construct
  REGION 1..10: note = Description of Artificial Sequence: Synthetic peptide
YSTDSSGNPV

SEQ ID NO: 345 - protein, 132 aa, synthetic construct
  REGION 1..132: note = Description of Artificial Sequence: Synthetic polypeptide
EVQLLESGGGLVQPGGSLRLSCAASGFTFSSYAMSWVRQAPGKGLEWVSAISGSGGSTYYADSVKGRFTISRDNSKNTLYLQMNSLRAEDTAVYYCAKIPWGDYDFWSGYYTRPGHSGMDVWGQGTLVTVSS

SEQ ID NO: 346 - protein, 108 aa, synthetic construct
  REGION 1..108: note = Description of Artificial Sequence: Synthetic polypeptide
SYELTQPPSVSVSPGQTARITCSGDALPKKYAYWYQQKSGQAPVLVIYEDSKRPSGIPERFSGSSSGTMATLTVSGAQVEDEADYYCYSTDSSGNPVFGGGTKLTVLG

SEQ ID NO: 347 - protein, 7 aa, synthetic construct
  REGION 1..7: note = Description of Artificial Sequence: Synthetic peptide
GFTFRAY

SEQ ID NO: 348 - protein, 10 aa, synthetic construct
  REGION 1..10: note = Description of Artificial Sequence: Synthetic peptide
GFTFRAYPMS

SEQ ID NO: 349 - protein, 5 aa, synthetic construct
  REGION 1..5: note = Description of Artificial Sequence: Synthetic peptide
AYPMS

SEQ ID NO: 350 - protein, 6 aa, synthetic construct
  REGION 1..6: note = Description of Artificial Sequence: Synthetic peptide
RAYPMS

SEQ ID NO: 351 - protein, 8 aa, synthetic construct
  REGION 1..8: note = Description of Artificial Sequence: Synthetic peptide
GFTFRAYP

SEQ ID NO: 352 - protein, 4 aa, synthetic construct
  REGION 1..4: note = Description of Artificial Sequence: Synthetic peptide
TSSG

SEQ ID NO: 353 - protein, 8 aa, synthetic construct
  REGION 1..8: note = Description of Artificial Sequence: Synthetic peptide
SITSSGSY

SEQ ID NO: 354 - protein, 15 aa, synthetic construct
  REGION 1..15: note = Description of Artificial Sequence: Synthetic peptide
SITSSGSYYADSVKG

SEQ ID NO: 355 - protein, 11 aa, synthetic construct
  REGION 1..11: note = Description of Artificial Sequence: Synthetic peptide
WVSSITSSGSY

SEQ ID NO: 356 - protein, 6 aa, synthetic construct
  REGION 1..6: note = Description of Artificial Sequence: Synthetic peptide
ITSSGS

SEQ ID NO: 357 - protein, 8 aa, synthetic construct
  REGION 1..8: note = Description of Artificial Sequence: Synthetic peptide
VGVTDFDY

SEQ ID NO: 358 - protein, 9 aa, synthetic construct
  REGION 1..9: note = Description of Artificial Sequence: Synthetic peptide
ARVGVTDFD

SEQ ID NO: 359 - protein, 10 aa, synthetic construct
  REGION 1..10: note = Description of Artificial Sequence: Synthetic peptide
ARVGVTDFDY

SEQ ID NO: 360 - protein, 14 aa, synthetic construct
  REGION 1..14: note = Description of Artificial Sequence: Synthetic peptide
AGSSSNIGAGYDVH

SEQ ID NO: 361 - protein, 10 aa, synthetic construct
  REGION 1..10: note = Description of Artificial Sequence: Synthetic peptide
IGAGYDVHWY

SEQ ID NO: 362 - protein, 9 aa, synthetic construct
  REGION 1..9: note = Description of Artificial Sequence: Synthetic peptide
SSNIGAGYD

SEQ ID NO: 363 - protein, 7 aa, synthetic construct
  REGION 1..7: note = Description of Artificial Sequence: Synthetic peptide
DSSNRPS

SEQ ID NO: 364 - protein, 10 aa, synthetic construct
  REGION 1..10: note = Description of Artificial Sequence: Synthetic peptide
LLIFDSSNRP

SEQ ID NO: 365 - protein, 12 aa, synthetic construct
  REGION 1..12: note = Description of Artificial Sequence: Synthetic peptide
QSYDFRLSGSMV

SEQ ID NO: 366 - protein, 115 aa, synthetic construct
  REGION 1..115: note = Description of Artificial Sequence: Synthetic polypeptide
EVQLVESGGGLVKPGGSLRLSCAASGFTFRAYPMSWVRQAPGKGLEWVSSITSSGSYYADSVKGRFTISRDNAKSSLYLQMNSLRADDTAVYYCARVGVTDFDYWGQGTLVTVSS

SEQ ID NO: 367 - protein, 113 aa, synthetic construct
  REGION 1..113: note = Description of Artificial Sequence: Synthetic polypeptide
QAVLTQPPSVSGAPGQRVTISCAGSSSNIGAGYDVHWYQQLPGTAPKLLIFDSSNRPSGVPDRFSGSKSGTSASLAITGLQAEDEADYYCQSYDFRLSGSMVFGGGTKLTVLG

SEQ ID NO: 368 - protein, 11 aa, synthetic construct
  REGION 1..11: note = Description of Artificial Sequence: Synthetic peptide
SIRTGSGYFDY

SEQ ID NO: 369 - protein, 12 aa, synthetic construct
  REGION 1..12: note = Description of Artificial Sequence: Synthetic peptide
AKSIRTGSGYFD

SEQ ID NO: 370 - protein, 13 aa, synthetic construct
  REGION 1..13: note = Description of Artificial Sequence: Synthetic peptide
SGSSSNIGTNYVY

SEQ ID NO: 371 - protein, 9 aa, synthetic construct
  REGION 1..9: note = Description of Artificial Sequence: Synthetic peptide
IGTNYVYWY

SEQ ID NO: 372 - protein, 8 aa, synthetic construct
  REGION 1..8: note = Description of Artificial Sequence: Synthetic peptide
SSNIGTNY

SEQ ID NO: 373 - protein, 7 aa, synthetic construct
  REGION 1..7: note = Description of Artificial Sequence: Synthetic peptide
RNNQRPS

SEQ ID NO: 374 - protein, 10 aa, synthetic construct
  REGION 1..10: note = Description of Artificial Sequence: Synthetic peptide
LLIYRNNQRP

SEQ ID NO: 375 - protein, 11 aa, synthetic construct
  REGION 1..11: note = Description of Artificial Sequence: Synthetic peptide
AAWDDSLSGWV

SEQ ID NO: 376 - protein, 120 aa, synthetic construct
  REGION 1..120: note = Description of Artificial Sequence: Synthetic polypeptide
EVQLLESGGGLVQPGGSLRLSCAASGFTFSSYAMSWVRQAPGKGLEWVSAISGSGGSTYYADSVKGRFTISRDNSKNTLYLQMNSLRAEDTAVYYCAKSIRTGSGYFDYWGQGTLVTVSS

SEQ ID NO: 377 - protein, 111 aa, synthetic construct
  REGION 1..111: note = Description of Artificial Sequence: Synthetic polypeptide
QSVLTQPPSASGTPGQRVTISCSGSSSNIGTNYVYWYQQLPGTAPKLLIYRNNQRPSGAPDRFSGSKSGTSASLAISGLRSEDEADYYCAAWDDSLSGWVFGGGTKVTVLG

SEQ ID NO: 378 - protein, 7 aa, synthetic construct
  REGION 1..7: note = Description of Artificial Sequence: Synthetic peptide
GYTFTSY

SEQ ID NO: 379 - protein, 10 aa, synthetic construct
  REGION 1..10: note = Description of Artificial Sequence: Synthetic peptide
GYTFTSYYMH

SEQ ID NO: 380 - protein, 5 aa, synthetic construct
  REGION 1..5: note = Description of Artificial Sequence: Synthetic peptide
SYYMH

SEQ ID NO: 381 - protein, 6 aa, synthetic construct
  REGION 1..6: note = Description of Artificial Sequence: Synthetic peptide
TSYYMH

SEQ ID NO: 382 - protein, 8 aa, synthetic construct
  REGION 1..8: note = Description of Artificial Sequence: Synthetic peptide
GYTFTSYY

SEQ ID NO: 383 - protein, 6 aa, synthetic construct
  REGION 1..6: note = Description of Artificial Sequence: Synthetic peptide
NPSGGS

SEQ ID NO: 384 - protein, 10 aa, synthetic construct
  REGION 1..10: note = Description of Artificial Sequence: Synthetic peptide
IINPSGGSTS

SEQ ID NO: 385 - protein, 13 aa, synthetic construct
  REGION 1..13: note = Description of Artificial Sequence: Synthetic peptide
WMGIINPSGGSTS

SEQ ID NO: 386 - protein, 8 aa, synthetic construct
  REGION 1..8: note = Description of Artificial Sequence: Synthetic peptide
INPSGGST

SEQ ID NO: 387 - protein, 13 aa, synthetic construct
  REGION 1..13: note = Description of Artificial Sequence: Synthetic peptide
DLLLYGRGGGFQH

SEQ ID NO: 388 - protein, 14 aa, synthetic construct
  REGION 1..14: note = Description of Artificial Sequence: Synthetic peptide
ARDLLLYGRGGGFQ

SEQ ID NO: 389 - protein, 15 aa, synthetic construct
  REGION 1..15: note = Description of Artificial Sequence: Synthetic peptide
ARDLLLYGRGGGFQH

SEQ ID NO: 390 - protein, 9 aa, synthetic construct
  REGION 1..9: note = Description of Artificial Sequence: Synthetic peptide
IGSNYVYWY

SEQ ID NO: 391 - protein, 8 aa, synthetic construct
  REGION 1..8: note = Description of Artificial Sequence: Synthetic peptide
SSNIGSNY

SEQ ID NO: 392 - protein, 121 aa, synthetic construct
  REGION 1..121: note = Description of Artificial Sequence: Synthetic polypeptide
QVQLQSGAEVKKPGASVKVSCKASGYTFTSYYMHWVRQAPGQGLEWMGIINPSGGSTSYAQKFQGRVTMTRDTSTSTVYMELSSLRSEDTAVYYCARDLLLYGRGGGFQHWGQGTLVTVSS

SEQ ID NO: 393 - protein, 111 aa, synthetic construct
  REGION 1..111: note = Description of Artificial Sequence: Synthetic polypeptide
QSVLTQPPSASGTPGQRVTISCSGSSSNIGSNYVYWYQQLPGTAPKLLIYRNNQRPSGVPDRFSGSKSGTSASLAISGLRSEDEADYYCAAWDDSLSGWVFGGGTKLTVLG

SEQ ID NO: 394 - protein, 7 aa, synthetic construct
  REGION 1..7: note = Description of Artificial Sequence: Synthetic peptide
GFTFDDY

SEQ ID NO: 395 - protein, 10 aa, synthetic construct
  REGION 1..10: note = Description of Artificial Sequence: Synthetic peptide
GFTFDDYGMS

SEQ ID NO: 396 - protein, 5 aa, synthetic construct
  REGION 1..5: note = Description of Artificial Sequence: Synthetic peptide
DYGMS

SEQ ID NO: 397 - protein, 6 aa, synthetic construct
  REGION 1..6: note = Description of Artificial Sequence: Synthetic peptide
DDYGMS

SEQ ID NO: 398 - protein, 8 aa, synthetic construct
  REGION 1..8: note = Description of Artificial Sequence: Synthetic peptide
GFTFDDYG

SEQ ID NO: 399 - protein, 6 aa, synthetic construct
  REGION 1..6: note = Description of Artificial Sequence: Synthetic peptide
NWNGGS

SEQ ID NO: 400 - protein, 10 aa, synthetic construct
  REGION 1..10: note = Description of Artificial Sequence: Synthetic peptide
GINWNGGSTG

SEQ ID NO: 401 - protein, 17 aa, synthetic construct
  REGION 1..17: note = Description of Artificial Sequence: Synthetic peptide
GINWNGGSTGYADSVKG

SEQ ID NO: 402 - protein, 13 aa, synthetic construct
  REGION 1..13: note = Description of Artificial Sequence: Synthetic peptide
WVSGINWNGGSTG

SEQ ID NO: 403 - protein, 8 aa, synthetic construct
  REGION 1..8: note = Description of Artificial Sequence: Synthetic peptide
INWNGGST

SEQ ID NO: 404 - protein, 6 aa, synthetic construct
  REGION 1..6: note = Description of Artificial Sequence: Synthetic peptide
KSTGDY

SEQ ID NO: 405 - protein, 7 aa, synthetic construct
  REGION 1..7: note = Description of Artificial Sequence: Synthetic peptide
ARKSTGD

SEQ ID NO: 406 - protein, 8 aa, synthetic construct
  REGION 1..8: note = Description of Artificial Sequence: Synthetic peptide
ARKSTGDY

SEQ ID NO: 407 - protein, 11 aa, synthetic construct
  REGION 1..11: note = Description of Artificial Sequence: Synthetic peptide
QGDSLRSYYAS

SEQ ID NO: 408 - protein, 7 aa, synthetic construct
  REGION 1..7: note = Description of Artificial Sequence: Synthetic peptide
SYYASWY

SEQ ID NO: 409 - protein, 6 aa, synthetic construct
  REGION 1..6: note = Description of Artificial Sequence: Synthetic peptide
SLRSYY

SEQ ID NO: 410 - protein, 7 aa, synthetic construct
  REGION 1..7: note = Description of Artificial Sequence: Synthetic peptide
GKNNRPS

SEQ ID NO: 411 - protein, 10 aa, synthetic construct
  REGION 1..10: note = Description of Artificial Sequence: Synthetic peptide
LVIYGKNNRP

SEQ ID NO: 412 - protein, 12 aa, synthetic construct
  REGION 1..12: note = Description of Artificial Sequence: Synthetic peptide
NSRDNSGKHLWV

SEQ ID NO: 413 - protein, 115 aa, synthetic construct
  REGION 1..115: note = Description of Artificial Sequence: Synthetic polypeptide
EVQLVQSGGGVVRPGGSLRLSCAASGFTFDDYGMSWVRQAPGKGLEWVSGINWNGGSTGYADSVKGRFTISTDNAKNSLYLQMNSLRAEDTALYYCARKSTGDYWGQGTLVTVSS

SEQ ID NO: 414 - protein, 110 aa, synthetic construct
  REGION 1..110: note = Description of Artificial Sequence: Synthetic polypeptide
SSELTQDPAVSVALGQTVRITCQGDSLRSYYASWYQQKPGQAPVLVIYGKNNRPSGIPARFSGSSSGNTASLTITGAQAEDEADYYCNSRDNSGKHLWVFGGGTKLTVLG

SEQ ID NO: 415 - protein, 7 aa, synthetic construct
  REGION 1..7: note = Description of Artificial Sequence: Synthetic peptide
GFTFSDY

SEQ ID NO: 416 - protein, 10 aa, synthetic construct
  REGION 1..10: note = Description of Artificial Sequence: Synthetic peptide
GFTFSDYYMS

SEQ ID NO: 417 - protein, 5 aa, synthetic construct
  REGION 1..5: note = Description of Artificial Sequence: Synthetic peptide
DYYMS

SEQ ID NO: 418 - protein, 6 aa, synthetic construct
  REGION 1..6: note = Description of Artificial Sequence: Synthetic peptide
SDYYMS

SEQ ID NO: 419 - protein, 8 aa, synthetic construct
  REGION 1..8: note = Description of Artificial Sequence: Synthetic peptide
GFTFSDYY

SEQ ID NO: 420 - protein, 6 aa, synthetic construct
  REGION 1..6: note = Description of Artificial Sequence: Synthetic peptide
SSSSSY

SEQ ID NO: 421 - protein, 10 aa, synthetic construct
  REGION 1..10: note = Description of Artificial Sequence: Synthetic peptide
YISSSSSYTN

SEQ ID NO: 422 - protein, 17 aa, synthetic construct
  REGION 1..17: note = Description of Artificial Sequence: Synthetic peptide
YISSSSSYTNYADSVKG

SEQ ID NO: 423 - protein, 13 aa, synthetic construct
  REGION 1..13: note = Description of Artificial Sequence: Synthetic peptide
WVSYISSSSSYTN

SEQ ID NO: 424 - protein, 8 aa, synthetic construct
  REGION 1..8: note = Description of Artificial Sequence: Synthetic peptide
ISSSSSYT

SEQ ID NO: 425 - protein, 9 aa, synthetic construct
  REGION 1..9: note = Description of Artificial Sequence: Synthetic peptide
VNYYYGMDV

SEQ ID NO: 426 - protein, 10 aa, synthetic construct
  REGION 1..10: note = Description of Artificial Sequence: Synthetic peptide
ARVNYYYGMD

SEQ ID NO: 427 - protein, 11 aa, synthetic construct
  REGION 1..11: note = Description of Artificial Sequence: Synthetic peptide
ARVNYYYGMDV

SEQ ID NO: 428 - protein, 10 aa, synthetic construct
  REGION 1..10: note = Description of Artificial Sequence: Synthetic peptide
LLIYGNSNRP

SEQ ID NO: 429 - protein, 13 aa, synthetic construct
  REGION 1..13: note = Description of Artificial Sequence: Synthetic peptide
AAWDDSLNGPRMV

SEQ ID NO: 430 - protein, 118 aa, synthetic construct
  REGION 1..118: note = Description of Artificial Sequence: Synthetic polypeptide
EVQLVQSGGGLVKPGGSLRLSCAASGFTFSDYYMSWIRQAPGKGLEWVSYISSSSSYTNYADSVKGRFTISRDNAKNSLYLQMNSLRAEDTAVYYCARVNYYYGMDVWGQGTLVTVSS

SEQ ID NO: 431 - protein, 114 aa, synthetic construct
  REGION 1..114: note = Description of Artificial Sequence: Synthetic polypeptide
QSVLTQPPSVSGAPGQRVTISCTGSSSNIGAGYDVHWYQQLPGTAPKLLIYGNSNRPSGVPDRFSGSKSGTSASLAISGLQSEDEADYYCAAWDDSLNGPRMVFGGGTKLTVLG

SEQ ID NO: 432 - protein, 9 aa, synthetic construct
  REGION 1..9: note = Description of Artificial Sequence: Synthetic peptide
GGSISSGGY

SEQ ID NO: 433 - protein, 10 aa, synthetic construct
  REGION 1..10: note = Description of Artificial Sequence: Synthetic peptide
GGSISSGGYY

SEQ ID NO: 434 - protein, 9 aa, synthetic construct
  REGION 1..9: note = Description of Artificial Sequence: Synthetic peptide
YIYYSGSTY

SEQ ID NO: 435 - protein, 16 aa, synthetic construct
  REGION 1..16: note = Description of Artificial Sequence: Synthetic peptide
YIYYSGSTYYNPSLKG

SEQ ID NO: 436 - protein, 12 aa, synthetic construct
  REGION 1..12: note = Description of Artificial Sequence: Synthetic peptide
WIGYIYYSGSTY

SEQ ID NO: 437 - protein, 9 aa, synthetic construct
  REGION 1..9: note = Description of Artificial Sequence: Synthetic peptide
EEVGDWFDP

SEQ ID NO: 438 - protein, 10 aa, synthetic construct
  REGION 1..10: note = Description of Artificial Sequence: Synthetic peptide
AREEVGDWFD

SEQ ID NO: 439 - protein, 11 aa, synthetic construct
  REGION 1..11: note = Description of Artificial Sequence: Synthetic peptide
AREEVGDWFDP

SEQ ID NO: 440 - protein, 7 aa, synthetic construct
  REGION 1..7: note = Description of Artificial Sequence: Synthetic peptide
KYYASWY

SEQ ID NO: 441 - protein, 6 aa, synthetic construct
  REGION 1..6: note = Description of Artificial Sequence: Synthetic peptide
SLRKYY

SEQ ID NO: 442 - protein, 7 aa, synthetic construct
  REGION 1..7: note = Description of Artificial Sequence: Synthetic peptide
GKNKRPS

SEQ ID NO: 443 - protein, 10 aa, synthetic construct
  REGION 1..10: note = Description of Artificial Sequence: Synthetic peptide
LVIYGKNKRP

SEQ ID NO: 444 - protein, 119 aa, synthetic construct
  REGION 1..119: note = Description of Artificial Sequence: Synthetic polypeptide
QVQLQESGPGLVKPSQTLSLTCTVSGGSISSGGYYWSWIRQHPGKGLEWIGYIYYSGSTYYNPSLKGRVTISVDTSKNQFSLKLSSVTAADTAVYYCAREEVGDWFDPWGQGTLVTVSS

SEQ ID NO: 445 - protein, 109 aa, synthetic construct
  REGION 1..109: note = Description of Artificial Sequence: Synthetic polypeptide
SSELTQDPAVSVALGQTVRITCQGDSLRKYYASWYQQKAGQAPVLVIYGKNKRPSGIPDRFSGSSSGNTASLTITGAQAEDEADYYCNSWDSSGNHVVFGGGTKLTVLG

SEQ ID NO: 446 - protein, 6 aa, synthetic construct
  REGION 1..6: note = Description of Artificial Sequence: Synthetic peptide
NPNGGG

SEQ ID NO: 447 - protein, 10 aa, synthetic construct
  REGION 1..10: note = Description of Artificial Sequence: Synthetic peptide
WINPNGGGTK

SEQ ID NO: 448 - protein, 17 aa, synthetic construct
  REGION 1..17: note = Description of Artificial Sequence: Synthetic peptide
WINPNGGGTKYAQKFQG

SEQ ID NO: 449 - protein, 13 aa, synthetic construct
  REGION 1..13: note = Description of Artificial Sequence: Synthetic peptide
WMGWINPNGGGTK

SEQ ID NO: 450 - protein, 8 aa, synthetic construct
  REGION 1..8: note = Description of Artificial Sequence: Synthetic peptide
INPNGGGT

SEQ ID NO: 451 - protein, 9 aa, synthetic construct
  REGION 1..9: note = Description of Artificial Sequence: Synthetic peptide
LSDYSSGGP

SEQ ID NO: 452 - protein, 10 aa, synthetic construct
  REGION 1..10: note = Description of Artificial Sequence: Synthetic peptide
ATLSDYSSGG

SEQ ID NO: 453 - protein, 11 aa, synthetic construct
  REGION 1..11: note = Description of Artificial Sequence: Synthetic peptide
ATLSDYSSGGR

SEQ ID NO: 454 - protein, 11 aa, synthetic construct
  REGION 1..11: note = Description of Artificial Sequence: Synthetic peptide
AAWDDSLSGVV

SEQ ID NO: 455 - protein, 117 aa, synthetic construct
  REGION 1..117: note = Description of Artificial Sequence: Synthetic polypeptide
QVQLQSGAEVKKPGASVKVSCKASGYTFTGYYMHWVRQAPGQGLEWMGWINPNGGGTKYAQKFQGRVTMTRDTSISTAYMELSSLRSDDTAVYYCATLSDYSSGGPWGQGTLVTVSS

SEQ ID NO: 456 - protein, 111 aa, synthetic construct
  REGION 1..111: note = Description of Artificial Sequence: Synthetic polypeptide
QSVLTQPPSASGTPGQRVTISCSGSSSNIGSNYVYWYQQLPGTAPKLLIYRNNQRPSGVPDRFSGSKSGTSASLAISGLRSEDEADYYCAAWDDSLSGVVFGGGTKLTVLG

SEQ ID NO: 457 - protein, 10 aa, synthetic construct
  REGION 1..10: note = Description of Artificial Sequence: Synthetic peptide
GYTFTGYHVH

SEQ ID NO: 458 - protein, 5 aa, synthetic construct
  REGION 1..5: note = Description of Artificial Sequence: Synthetic peptide
GYHVH

SEQ ID NO: 459 - protein, 6 aa, synthetic construct
  REGION 1..6: note = Description of Artificial Sequence: Synthetic peptide
TGYHVH

SEQ ID NO: 460 - protein, 8 aa, synthetic construct
  REGION 1..8: note = Description of Artificial Sequence: Synthetic peptide
GYTFTGYH

SEQ ID NO: 461 - protein, 6 aa, synthetic construct
  REGION 1..6: note = Description of Artificial Sequence: Synthetic peptide
NPDSGG

SEQ ID NO: 462 - protein, 10 aa, synthetic construct
  REGION 1..10: note = Description of Artificial Sequence: Synthetic peptide
WINPDSGGTN

SEQ ID NO: 463 - protein, 17 aa, synthetic construct
  REGION 1..17: note = Description of Artificial Sequence: Synthetic peptide
WINPDSGGTNFAQKFQG

SEQ ID NO: 464 - protein, 13 aa, synthetic construct
  REGION 1..13: note = Description of Artificial Sequence: Synthetic peptide
WMGWINPDSGGTN

SEQ ID NO: 465 - protein, 8 aa, synthetic construct
  REGION 1..8: note = Description of Artificial Sequence: Synthetic peptide
INPDSGGT

SEQ ID NO: 466 - protein, 5 aa, synthetic construct
  REGION 1..5: note = Description of Artificial Sequence: Synthetic peptide
RSLDY

SEQ ID NO: 467 - protein, 6 aa, synthetic construct
  REGION 1..6: note = Description of Artificial Sequence: Synthetic peptide
ARRSLD

SEQ ID NO: 468 - protein, 7 aa, synthetic construct
  REGION 1..7: note = Description of Artificial Sequence: Synthetic peptide
ARRSLDY

SEQ ID NO: 469 - protein, 114 aa, synthetic construct
  REGION 1..114: note = Description of Artificial Sequence: Synthetic polypeptide
EVQLVQSGTEVKRPGASVKVSCKASGYTFTGYHVHWVRQAPGQGLEWMGWINPDSGGTNFAQKFQGRVTMTRDTSISTAYMELTSLRSDDTAIYYCARRSLDYWGQGTLVTVSS

SEQ ID NO: 470 - protein, 111 aa, synthetic construct
  REGION 1..111: note = Description of Artificial Sequence: Synthetic polypeptide
QAVLTQPPSASGTPGQRVTISCSGSSSNIGSNYVYWYQQLPGTAPKLLIYRNNQRPSGVPDRFSGSKSGTSASLAISGLRSEDEADYYCAAWDDSLSGVVFGGGTKLTVLG

SEQ ID NO: 471 - protein, 7 aa, synthetic construct
  REGION 1..7: note = Description of Artificial Sequence: Synthetic peptide
GFTFSNA

SEQ ID NO: 472 - protein, 10 aa, synthetic construct
  REGION 1..10: note = Description of Artificial Sequence: Synthetic peptide
GFTFSNAWMS

SEQ ID NO: 473 - protein, 5 aa, synthetic construct
  REGION 1..5: note = Description of Artificial Sequence: Synthetic peptide
NAWMS

SEQ ID NO: 474 - protein, 6 aa, synthetic construct
  REGION 1..6: note = Description of Artificial Sequence: Synthetic peptide
SNAWMS

SEQ ID NO: 475 - protein, 8 aa, synthetic construct
  REGION 1..8: note = Description of Artificial Sequence: Synthetic peptide
GFTFSNAW

SEQ ID NO: 476 - protein, 8 aa, synthetic construct
  REGION 1..8: note = Description of Artificial Sequence: Synthetic peptide
KSKTDGGT

SEQ ID NO: 477 - protein, 12 aa, synthetic construct
  REGION 1..12: note = Description of Artificial Sequence: Synthetic peptide
RIKSKTDGGTTD

SEQ ID NO: 478 - protein, 19 aa, synthetic construct
  REGION 1..19: note = Description of Artificial Sequence: Synthetic peptide
RIKSKTDGGTTDYAAPVKG

SEQ ID NO: 479 - protein, 15 aa, synthetic construct
  REGION 1..15: note = Description of Artificial Sequence: Synthetic peptide
WVGRIKSKTDGGTTD

SEQ ID NO: 480 - protein, 10 aa, synthetic construct
  REGION 1..10: note = Description of Artificial Sequence: Synthetic peptide
IKSKTDGGTT

SEQ ID NO: 481 - protein, 4 aa, synthetic construct
  REGION 1..4: note = Description of Artificial Sequence: Synthetic peptide
LVDY

SEQ ID NO: 482 - protein, 5 aa, synthetic construct
  REGION 1..5: note = Description of Artificial Sequence: Synthetic peptide
ASLVD

SEQ ID NO: 483 - protein, 115 aa, synthetic construct
  REGION 1..115: note = Description of Artificial Sequence: Synthetic polypeptide
EVQLVQSGGGLVQPGGSLRLSCAASGFTFSNAWMSWVRQAPGKGLEWVGRIKSKTDGGTTDYAAPVKGRFTISRDDSKNTLYLQMNSLKTEDTAVYYCASLVDYWGQGTLVTVSS

SEQ ID NO: 484 - protein, 111 aa, synthetic construct
  REGION 1..111: note = Description of Artificial Sequence: Synthetic polypeptide
SYELTQPPSASGTPGQRVTISCSGSSSNIGSNYVYWYQQLPGTAPKLLIYRNNQRPSGVPDRFSASKSGTSASLAISGLQSADEADYYCAAWDDSLNGVVFGGGTKLTVLG

SEQ ID NO: 485 - protein, 7 aa, synthetic construct
  REGION 1..7: note = Description of Artificial Sequence: Synthetic peptide
GYTFTKY

SEQ ID NO: 486 - protein, 10 aa, synthetic construct
  REGION 1..10: note = Description of Artificial Sequence: Synthetic peptide
GYTFTKYGIS

SEQ ID NO: 487 - protein, 5 aa, synthetic construct
  REGION 1..5: note = Description of Artificial Sequence: Synthetic peptide
KYGIS

SEQ ID NO: 488 - protein, 6 aa, synthetic construct
  REGION 1..6: note = Description of Artificial Sequence: Synthetic peptide
TKYGIS

SEQ ID NO: 489 - protein, 8 aa, synthetic construct
  REGION 1..8: note = Description of Artificial Sequence: Synthetic peptide
GYTFTKYG

SEQ ID NO: 490 - protein, 6 aa, synthetic construct
  REGION 1..6: note = Description of Artificial Sequence: Synthetic peptide
SAYNVD

SEQ ID NO: 491 - protein, 10 aa, synthetic construct
  REGION 1..10: note = Description of Artificial Sequence: Synthetic peptide
WISAYNVDTK

SEQ ID NO: 492 - protein, 17 aa, synthetic construct
  REGION 1..17: note = Description of Artificial Sequence: Synthetic peptide
WISAYNVDTKYAQKFQG

SEQ ID NO: 493 - protein, 13 aa, synthetic construct
  REGION 1..13: note = Description of Artificial Sequence: Synthetic peptide
WMGWISAYNVDTK

SEQ ID NO: 494 - protein, 8 aa, synthetic construct
  REGION 1..8: note = Description of Artificial Sequence: Synthetic peptide
ISAYNVDT

SEQ ID NO: 495 - protein, 5 aa, synthetic construct
  REGION 1..5: note = Description of Artificial Sequence: Synthetic peptide
RGLDY

SEQ ID NO: 496 - protein, 6 aa, synthetic construct
  REGION 1..6: note = Description of Artificial Sequence: Synthetic peptide
ARRGLD

SEQ ID NO: 497 - protein, 7 aa, synthetic construct
  REGION 1..7: note = Description of Artificial Sequence: Synthetic peptide
ARRGLDY

SEQ ID NO: 498 - protein, 11 aa, synthetic construct
  REGION 1..11: note = Description of Artificial Sequence: Synthetic peptide
AAWDDSLSGPV

SEQ ID NO: 499 - protein, 114 aa, synthetic construct
  REGION 1..114: note = Description of Artificial Sequence: Synthetic polypeptide
EVQLVQSGAVVKKPGASVKVSCKASGYTFTKYGISWVRQAPEQGLEWMGWISAYNVDTKYAQKFQGRVTMTTDTSTSTAYMELRSLRSDDTAVYYCARRGLDYWGQGTLVTVSS

SEQ ID NO: 500 - protein, 111 aa, synthetic construct
  REGION 1..111: note = Description of Artificial Sequence: Synthetic polypeptide
QSVLTQPPSASGTPGQRVTISCSGSSSNIGSNYVYWYQQLPGTAPKLLIYRNNQRPSGVPDRFSGSKSGTSASLAISGLRSEDEADYYCAAWDDSLSGPVFGGGTKVTVLG

SEQ ID NO: 501 - protein, 7 aa, synthetic construct
  REGION 1..7: note = Description of Artificial Sequence: Synthetic peptide
GKSKRPS

SEQ ID NO: 502 - protein, 10 aa, synthetic construct
  REGION 1..10: note = Description of Artificial Sequence: Synthetic peptide
LVIYGKSKRP

SEQ ID NO: 503 - protein, 7 aa, synthetic construct
  REGION 1..7: note = Description of Artificial Sequence: Synthetic peptide
GGTFSSY

SEQ ID NO: 504 - protein, 10 aa, synthetic construct
  REGION 1..10: note = Description of Artificial Sequence: Synthetic peptide
GGTFSSYAIS

SEQ ID NO: 505 - protein, 5 aa, synthetic construct
  REGION 1..5: note = Description of Artificial Sequence: Synthetic peptide
SYAIS

SEQ ID NO: 506 - protein, 6 aa, synthetic construct
  REGION 1..6: note = Description of Artificial Sequence: Synthetic peptide
SSYAIS

SEQ ID NO: 507 - protein, 8 aa, synthetic construct
  REGION 1..8: note = Description of Artificial Sequence: Synthetic peptide
GGTFSSYA

SEQ ID NO: 508 - protein, 6 aa, synthetic construct
  REGION 1..6: note = Description of Artificial Sequence: Synthetic peptide
IPILGI

SEQ ID NO: 509 - protein, 10 aa, synthetic construct
  REGION 1..10: note = Description of Artificial Sequence: Synthetic peptide
RIIPILGIAN

SEQ ID NO: 510 - protein, 17 aa, synthetic construct
  REGION 1..17: note = Description of Artificial Sequence: Synthetic peptide
RIIPILGIANYAQKFQG

SEQ ID NO: 511 - protein, 13 aa, synthetic construct
  REGION 1..13: note = Description of Artificial Sequence: Synthetic peptide
WMGRIIPILGIAN

SEQ ID NO: 512 - protein, 8 aa, synthetic construct
  REGION 1..8: note = Description of Artificial Sequence: Synthetic peptide
IIPILGIA

SEQ ID NO: 513 - protein, 8 aa, synthetic construct
  REGION 1..8: note = Description of Artificial Sequence: Synthetic peptide
DLWGVGAD

SEQ ID NO: 514 - protein, 9 aa, synthetic construct
  REGION 1..9: note = Description of Artificial Sequence: Synthetic peptide
ATDLWGVGA

SEQ ID NO: 515 - protein, 10 aa, synthetic construct
  REGION 1..10: note = Description of Artificial Sequence: Synthetic peptide
ATDLWGVGAD

SEQ ID NO: 516 - protein, 14 aa, synthetic construct
  REGION 1..14: note = Description of Artificial Sequence: Synthetic peptide
TGTSSDVGGYKSVS

SEQ ID NO: 517 - protein, 10 aa, synthetic construct
  REGION 1..10: note = Description of Artificial Sequence: Synthetic peptide
VGGYKSVSWY

SEQ ID NO: 518 - protein, 9 aa, synthetic construct
  REGION 1..9: note = Description of Artificial Sequence: Synthetic peptide
SSDVGGYKS

SEQ ID NO: 519 - protein, 7 aa, synthetic construct
  REGION 1..7: note = Description of Artificial Sequence: Synthetic peptide
DVSNRPS

SEQ ID NO: 520 - protein, 10 aa, synthetic construct
  REGION 1..10: note = Description of Artificial Sequence: Synthetic peptide
LMIYDVSNRP

SEQ ID NO: 521 - protein, 11 aa, synthetic construct
  REGION 1..11: note = Description of Artificial Sequence: Synthetic peptide
SSYTSSSSLWV

SEQ ID NO: 522 - protein, 15 aa, synthetic construct
  REGION 1..15: note = Description of Artificial Sequence: Synthetic peptide
GGGGSGGGGSGDGSS

SEQ ID NO: 523 - protein, 121 aa, synthetic construct
  REGION 1..121: note = Description of Artificial Sequence: Synthetic polypeptide
EVQLVGSGGGVVQPGRSLRLSCAASGFTFSNYAMHWVRQAPGKGLEWVAVISYDGSNKYYADSVKGRFTISRDNSKNTLYLQMNSLRAEDTAVYYCARVRYYGSGSPIGYWGQGTLVTVSS

SEQ ID NO: 524 - protein, 112 aa, synthetic construct
  REGION 1..112: note = Description of Artificial Sequence: Synthetic polypeptide
QSALTQPASVSGSPGQSITISCTGTSSDVGGYKSVSWYQQHPGKAPKLMIYDVSNRPSGVSDRFSGSKSGNTASLTISGLQAEDEADYYCSSYTSSSSLWVFGGGTKLTVLG

SEQ ID NO: 525 - protein, 10 aa, synthetic construct
  REGION 1..10: note = Description of Artificial Sequence: Synthetic peptide
GFTFDDYAMH

SEQ ID NO: 526 - protein, 5 aa, synthetic construct
  REGION 1..5: note = Description of Artificial Sequence: Synthetic peptide
DYAMH

SEQ ID NO: 527 - protein, 6 aa, synthetic construct
  REGION 1..6: note = Description of Artificial Sequence: Synthetic peptide
DDYAMH

SEQ ID NO: 528 - protein, 8 aa, synthetic construct
  REGION 1..8: note = Description of Artificial Sequence: Synthetic peptide
GFTFDDYA

SEQ ID NO: 529 - protein, 6 aa, synthetic construct
  REGION 1..6: note = Description of Artificial Sequence: Synthetic peptide
SWNSGS

SEQ ID NO: 530 - protein, 10 aa, synthetic construct
  REGION 1..10: note = Description of Artificial Sequence: Synthetic peptide
GISWNSGSIG

SEQ ID NO: 531 - protein, 17 aa, synthetic construct
  REGION 1..17: note = Description of Artificial Sequence: Synthetic peptide
GISWNSGSIGYADSVKG

SEQ ID NO: 532 - protein, 13 aa, synthetic construct
  REGION 1..13: note = Description of Artificial Sequence: Synthetic peptide
WVSGISWNSGSIG

SEQ ID NO: 533 - protein, 8 aa, synthetic construct
  REGION 1..8: note = Description of Artificial Sequence: Synthetic peptide
ISWNSGSI

SEQ ID NO: 534 - protein, 15 aa, synthetic construct
  REGION 1..15: note = Description of Artificial Sequence: Synthetic peptide
GGWGSSTHYYYGMDV

SEQ ID NO: 535 - protein, 16 aa, synthetic construct
  REGION 1..16: note = Description of Artificial Sequence: Synthetic peptide
AKGGWGSSTHYYYGMD

SEQ ID NO: 536 - protein, 17 aa, synthetic construct
  REGION 1..17: note = Description of Artificial Sequence: Synthetic peptide
AKGGWGSSTHYYYGMDV

SEQ ID NO: 537 - protein, 10 aa, synthetic construct
  REGION 1..10: note = Description of Artificial Sequence: Synthetic peptide
NVATYRIYWY

SEQ ID NO: 538 - protein, 9 aa, synthetic construct
  REGION 1..9: note = Description of Artificial Sequence: Synthetic peptide
SGINVATYR

SEQ ID NO: 539 - protein, 14 aa, synthetic construct
  REGION 1..14: note = Description of Artificial Sequence: Synthetic peptide
YLLTYKSDLDKHQG

SEQ ID NO: 540 - protein, 6 aa, synthetic construct
  REGION 1..6: note = Description of Artificial Sequence: Synthetic peptide
YKSDLD

SEQ ID NO: 541 - protein, 8 aa, synthetic construct
  REGION 1..8: note = Description of Artificial Sequence: Synthetic peptide
LIWHDYVW

SEQ ID NO: 542 - protein, 162 aa, synthetic construct
  REGION 1..162: note = Description of Artificial Sequence: Synthetic polypeptide
  MOD_RES 151: note = Any amino acid
  MOD_RES 155: note = Any amino acid
EVQLLESGGGLVQPGRSLRLSCAASGFTFDDYAMHWVRQAPGKGLEWVSGISWNSGSIGYADSVKGRFTISRDNAKNSLYLQMNSLRAEDTALYYCAKGGWGSSTHYYYGMDVWGQGTTVTVSSVDPFVSEYQGQSSDLPQPPVNAGGGSXGGGXRWWLWFR

SEQ ID NO: 543 - protein, 122 aa, synthetic construct
  REGION 1..122: note = Description of Artificial Sequence: Synthetic polypeptide
DDDDKLQAVLTQPSSLSASPGASASLTCTLHSGINVATYRIYWYQQKPGSPPQYLLTYKSDLDKHQGSGVPSRFSGSKDASANAGILLISGLQSDDEGDYYCLIWHDYVWYFGGGTKVTVLG

SEQ ID NO: 544 - protein, 9 aa, synthetic construct
  REGION 1..9: note = Description of Artificial Sequence: Synthetic peptide
GGSISSDDY

SEQ ID NO: 545 - protein, 12 aa, synthetic construct
  REGION 1..12: note = Description of Artificial Sequence: Synthetic peptide
GGSISSDDYYWS

SEQ ID NO: 546 - protein, 7 aa, synthetic construct
  REGION 1..7: note = Description of Artificial Sequence: Synthetic peptide
SDDYYWS

SEQ ID NO: 547 - protein, 8 aa, synthetic construct
  REGION 1..8: note = Description of Artificial Sequence: Synthetic peptide
SSDDYYWS

SEQ ID NO: 548 - protein, 10 aa, synthetic construct
  REGION 1..10: note = Description of Artificial Sequence: Synthetic peptide
GGSISSDDYY

SEQ ID NO: 549 - protein, 5 aa, synthetic construct
  REGION 1..5: note = Description of Artificial Sequence: Synthetic peptide
YYSGI

SEQ ID NO: 550 - protein, 9 aa, synthetic construct
  REGION 1..9: note = Description of Artificial Sequence: Synthetic peptide
YIYYSGITY

SEQ ID NO: 551 - protein, 16 aa, synthetic construct
  REGION 1..16: note = Description of Artificial Sequence: Synthetic peptide
YIYYSGITYYNPSLKS

SEQ ID NO: 552 - protein, 12 aa, synthetic construct
  REGION 1..12: note = Description of Artificial Sequence: Synthetic peptide
WIGYIYYSGITY

SEQ ID NO: 553 - protein, 7 aa, synthetic construct
  REGION 1..7: note = Description of Artificial Sequence: Synthetic peptide
IYYSGIT

SEQ ID NO: 554 - protein, 15 aa, synthetic construct
  REGION 1..15: note = Description of Artificial Sequence: Synthetic peptide
EGCNDGVCYNGVFDY

SEQ ID NO: 555 - protein, 16 aa, synthetic construct
  REGION 1..16: note = Description of Artificial Sequence: Synthetic peptide
AREGCNDGVCYNGVFD

SEQ ID NO: 556 - protein, 17 aa, synthetic construct
  REGION 1..17: note = Description of Artificial Sequence: Synthetic peptide
AREGCNDGVCYNGVFDY

SEQ ID NO: 557 - protein, 11 aa, synthetic construct
  REGION 1..11: note = Description of Artificial Sequence: Synthetic peptide
SGDKLGDKYAS

SEQ ID NO: 558 - protein, 7 aa, synthetic construct
  REGION 1..7: note = Description of Artificial Sequence: Synthetic peptide
DKYASWY

SEQ ID NO: 559 - protein, 6 aa, synthetic construct
  REGION 1..6: note = Description of Artificial Sequence: Synthetic peptide
KLGDKY

SEQ ID NO: 560 - protein, 7 aa, synthetic construct
  REGION 1..7: note = Description of Artificial Sequence: Synthetic peptide
QDSKRPS

SEQ ID NO: 561 - protein, 10 aa, synthetic construct
  REGION 1..10: note = Description of Artificial Sequence: Synthetic peptide
LVIYQDSKRP

SEQ ID NO: 562 - protein, 125 aa, synthetic construct
  REGION 1..125: note = Description of Artificial Sequence: Synthetic polypeptide
QVQLQESGPGLVKPSQTLSLTCTVSGGSISSDDYYWSWIRQTPGKGLEWIGYIYYSGITYYNPSLKSRVTISVDTSKNQFSLKLSSVTAADTAVYYCAREGCNDGVCYNGVFDYWGQGTLVTVSS

SEQ ID NO: 563 - protein, 107 aa, synthetic construct
  REGION 1..107: note = Description of Artificial Sequence: Synthetic polypeptide
SYELTQPPSMSVSPGQTASITCSGDKLGDKYASWYQQKPGQSPVLVIYQDSKRPSGIPERFSGSNSGNTATLTISGTQAMDEADYYCQAWDSSTAVFGGGTKLTVLG

SEQ ID NO: 564 - protein, 9 aa, synthetic construct
  REGION 1..9: note = Description of Artificial Sequence: Synthetic peptide
GDSIGSGDY

SEQ ID NO: 565 - protein, 12 aa, synthetic construct
  REGION 1..12: note = Description of Artificial Sequence: Synthetic peptide
GDSIGSGDYYWS

SEQ ID NO: 566 - protein, 7 aa, synthetic construct
  REGION 1..7: note = Description of Artificial Sequence: Synthetic peptide
SGDYYWS

SEQ ID NO: 567 - protein, 8 aa, synthetic construct
  REGION 1..8: note = Description of Artificial Sequence: Synthetic peptide
GSGDYYWS

SEQ ID NO: 568 - protein, 10 aa, synthetic construct
  REGION 1..10: note = Description of Artificial Sequence: Synthetic peptide
GDSIGSGDYY

SEQ ID NO: 569 - protein, 5 aa, synthetic construct
  REGION 1..5: note = Description of Artificial Sequence: Synthetic peptide
YHTGS

SEQ ID NO: 570 - protein, 9 aa, synthetic construct
  REGION 1..9: note = Description of Artificial Sequence: Synthetic peptide
YSYHTGSTD

SEQ ID NO: 571 - protein, 16 aa, synthetic construct
  REGION 1..16: note = Description of Artificial Sequence: Synthetic peptide
YSYHTGSTDYNPSLKS

SEQ ID NO: 572 - protein, 12 aa, synthetic construct
  REGION 1..12: note = Description of Artificial Sequence: Synthetic peptide
WIGYSYHTGSTD

SEQ ID NO: 573 - protein, 7 aa, synthetic construct
  REGION 1..7: note = Description of Artificial Sequence: Synthetic peptide
SYHTGST

SEQ ID NO: 574 - protein, 8 aa, synthetic construct
  REGION 1..8: note = Description of Artificial Sequence: Synthetic peptide
DYYGYLGY

SEQ ID NO: 575 - protein, 9 aa, synthetic construct
  REGION 1..9: note = Description of Artificial Sequence: Synthetic peptide
ARDYYGYLG

SEQ ID NO: 576 - protein, 10 aa, synthetic construct
  REGION 1..10: note = Description of Artificial Sequence: Synthetic peptide
ARDYYGYLGY

SEQ ID NO: 577 - protein, 14 aa, synthetic construct
  REGION 1..14: note = Description of Artificial Sequence: Synthetic peptide
AGTSSDVGTYNYVS

SEQ ID NO: 578 - protein, 10 aa, synthetic construct
  REGION 1..10: note = Description of Artificial Sequence: Synthetic peptide
VGTYNYVSWY

SEQ ID NO: 579 - protein, 9 aa, synthetic construct
  REGION 1..9: note = Description of Artificial Sequence: Synthetic peptide
SSDVGTYNY

SEQ ID NO: 580 - protein, 7 aa, synthetic construct
  REGION 1..7: note = Description of Artificial Sequence: Synthetic peptide
DVSKRPS

SEQ ID NO: 581 - protein, 10 aa, synthetic construct
  REGION 1..10: note = Description of Artificial Sequence: Synthetic peptide
LMIYDVSKRP

SEQ ID NO: 582 - protein, 10 aa, synthetic construct
  REGION 1..10: note = Description of Artificial Sequence: Synthetic peptide
YSYTTSSTWV

SEQ ID NO: 583 - protein, 118 aa, synthetic construct
  REGION 1..118: note = Description of Artificial Sequence: Synthetic polypeptide
QVQLQESGPGLLKPSQTLSLTCTVSGDSIGSGDYYWSWIRQPPGKGLEWIGYSYHTGSTDYNPSLKSRVSISVDRSKNQFSLKLRSVTAADTAVYYCARDYYGYLGYWGQGTLVTVSS

SEQ ID NO: 584 - protein, 111 aa, synthetic construct
  REGION 1..111: note = Description of Artificial Sequence: Synthetic polypeptide
QSALTQPASVSGSPGQSITISCAGTSSDVGTYNYVSWYQQHPGKAPKLMIYDVSKRPSGVPDRFSGSKSGNTASLTISGLQAEDEADYYCYSYTTSSTWVFGGGTKVTVLG

SEQ ID NO: 585 - protein, 11 aa, synthetic construct
  REGION 1..11: note = Description of Artificial Sequence: Synthetic peptide
RASQSISSYLN

SEQ ID NO: 586 - protein, 7 aa, synthetic construct
  REGION 1..7: note = Description of Artificial Sequence: Synthetic peptide
SSYLNWY

SEQ ID NO: 587 - protein, 6 aa, synthetic construct
  REGION 1..6: note = Description of Artificial Sequence: Synthetic peptide
QSISSY

SEQ ID NO: 588 - protein, 7 aa, synthetic construct
  REGION 1..7: note = Description of Artificial Sequence: Synthetic peptide
AASSLQS

SEQ ID NO: 589 - protein, 10 aa, synthetic construct
  REGION 1..10: note = Description of Artificial Sequence: Synthetic peptide
LLIYAASSLQ

SEQ ID NO: 590 - protein, 9 aa, synthetic construct
  REGION 1..9: note = Description of Artificial Sequence: Synthetic peptide
QQSYSTPRT

SEQ ID NO: 591 - protein, 107 aa, synthetic construct
  REGION 1..107: note = Description of Artificial Sequence: Synthetic polypeptide
DIQMTQSPSSLSASVGDRVTITCRASQSISSYLNWYQQKPGKAPKLLIYAASSLQSGVPSRFSGSGSGTDFTLTISSLQPEDFATYYCQQSYSTPRTFGQGTKVDIK

SEQ ID NO: 592 - protein, 7 aa, synthetic construct
  REGION 1..7: note = Description of Artificial Sequence: Synthetic peptide
GFTFSNY

SEQ ID NO: 593 - protein, 10 aa, synthetic construct
  REGION 1..10: note = Description of Artificial Sequence: Synthetic peptide
GFTFSNYAMH

SEQ ID NO: 594 - protein, 5 aa, synthetic construct
  REGION 1..5: note = Description of Artificial Sequence: Synthetic peptide
NYAMH

SEQ ID NO: 595 - protein, 6 aa, synthetic construct
  REGION 1..6: note = Description of Artificial Sequence: Synthetic peptide
SNYAMH

SEQ ID NO: 596 - protein, 8 aa, synthetic construct
  REGION 1..8: note = Description of Artificial Sequence: Synthetic peptide
GFTFSNYA

SEQ ID NO: 597 - protein, 6 aa, synthetic construct
  REGION 1..6: note = Description of Artificial Sequence: Synthetic peptide
SYDGSN

SEQ ID NO: 598 - protein, 10 aa, synthetic construct
  REGION 1..10: note = Description of Artificial Sequence: Synthetic peptide
VISYDGSNKY

SEQ ID NO: 599 - protein, 17 aa, synthetic construct
  REGION 1..17: note = Description of Artificial Sequence: Synthetic peptide
VISYDGSNKYYADSVKG

SEQ ID NO: 600 - protein, 13 aa, synthetic construct
  REGION 1..13: note = Description of Artificial Sequence: Synthetic peptide
WVAVISYDGSNKY

SEQ ID NO: 601 - protein, 8 aa, synthetic construct
  REGION 1..8: note = Description of Artificial Sequence: Synthetic peptide
ISYDGSNK

SEQ ID NO: 602 - protein, 12 aa, synthetic construct
  REGION 1..12: note = Description of Artificial Sequence: Synthetic peptide
VRYYGSGSPIGY

SEQ ID NO: 603 - protein, 13 aa, synthetic construct
  REGION 1..13: note = Description of Artificial Sequence: Synthetic peptide
ARVRYYGSGSPIG

SEQ ID NO: 604 - protein, 14 aa, synthetic construct
  REGION 1..14: note = Description of Artificial Sequence: Synthetic peptide
ARVRYYGSGSPIGY

SEQ ID NO: 605 - protein, 13 aa, synthetic construct
  REGION 1..13: note = Description of Artificial Sequence: Synthetic peptide
SGSSSNIGGNTVN

SEQ ID NO: 606 - protein, 9 aa, synthetic construct
  REGION 1..9: note = Description of Artificial Sequence: Synthetic peptide
IGGNTVNWY

SEQ ID NO: 607 - protein, 8 aa, synthetic construct
  REGION 1..8: note = Description of Artificial Sequence: Synthetic peptide
SSNIGGNT

SEQ ID NO: 608 - protein, 7 aa, synthetic construct
  REGION 1..7: note = Description of Artificial Sequence: Synthetic peptide
GDDLRPS

SEQ ID NO: 609 - protein, 10 aa, synthetic construct
  REGION 1..10: note = Description of Artificial Sequence: Synthetic peptide
LLIYGDDLRP

SEQ ID NO: 610 - protein, 11 aa, synthetic construct
  REGION 1..11: note = Description of Artificial Sequence: Synthetic peptide
AAWDDSLNAYV

SEQ ID NO: 611 - protein, 117 aa, synthetic construct
  REGION 1..117: note = Description of Artificial Sequence: Synthetic polypeptide
QVQLVQSGAEVKKPGSSVKVSCKASGGTFSSYAISWVRQAPGQGLEWMGRIIPILGIANYAQKFQGRVTMTEDTSTDTAYMELSSLRSEDTAVYYCATDLWGVGADWGQGTLVTVSS

SEQ ID NO: 612 - protein, 111 aa, synthetic construct
  REGION 1..111: note = Description of Artificial Sequence: Synthetic polypeptide
LPVLTQPPSASGTPGQRVTISCSGSSSNIGGNTVNWYHQLPGSAPKLLIYGDDLRPSGVPDRFSGSKSGTSASLAISRFQSGDEADYYCAAWDDSLNAYVFGTGTKLTVLG

SEQ ID NO: 613 - protein, 6 aa, synthetic construct
  REGION 1..6: note = Description of Artificial Sequence: Synthetic 6xHis tag
HHHHHH